European Patent Application EP 4 442 827 A1, published October 9, 2024. Title: 用于抑制乙型肝炎病毒（HBV）蛋白的表达的组合物和方法. Applicant: 上海舶望制药有限公司. The sequence listing filed with the application follows.

SEQUENCE LISTING (925 sequences)

SEQ ID NO: 1 - RNA, 21 nt, synthetic construct
  source 1..21: mol_type = other RNA
tggtggacttctctcaattta

SEQ ID NO: 2 - RNA, 21 nt, synthetic construct
  source 1..21: mol_type = other RNA
acttctctcaattttctagga

SEQ ID NO: 3 - RNA, 21 nt, synthetic construct
  source 1..21: mol_type = other RNA
gttaccaattttcttttgtca

SEQ ID NO: 4 - RNA, 21 nt, synthetic construct
  source 1..21: mol_type = other RNA
cataagaggactcttggacta

SEQ ID NO: 5 - RNA, 21 nt, synthetic construct
  source 1..21: mol_type = other RNA
ggggtttttcttgttgacaaa

SEQ ID NO: 6 - RNA, 21 nt, synthetic construct
  source 1..21: mol_type = other RNA
tggacttctctcaattttcta

SEQ ID NO: 7 - RNA, 21 nt, synthetic construct
  source 1..21: mol_type = other RNA
ctgctatgcctcatcttctta

SEQ ID NO: 8 - RNA, 21 nt, synthetic construct
  source 1..21: mol_type = other RNA
catttgttcagtggttcgtaa

SEQ ID NO: 9 - RNA, 21 nt, synthetic construct
  source 1..21: mol_type = other RNA
gggcgcacctctctttacgca

SEQ ID NO: 10 - RNA, 21 nt, synthetic construct
  source 1..21: mol_type = other RNA
tagactcgtggtggacttcta

SEQ ID NO: 11 - RNA, 21 nt, synthetic construct
  source 1..21: mol_type = other RNA
ggacttctctcaattttctaa

SEQ ID NO: 12 - RNA, 21 nt, synthetic construct
  source 1..21: mol_type = other RNA
ttggctcagtttactagtgca

SEQ ID NO: 13 - RNA, 21 nt, synthetic construct
  source 1..21: mol_type = other RNA
ctagtgccatttgttcagtga

SEQ ID NO: 14 - RNA, 21 nt, synthetic construct
  source 1..21: mol_type = other RNA
tgttaccaattttcttttgta

SEQ ID NO: 15 - RNA, 21 nt, synthetic construct
  source 1..21: mol_type = other RNA
ttcgcttcacctctgcacgta

SEQ ID NO: 16 - RNA, 21 nt, synthetic construct
  source 1..21: mol_type = other RNA
taggaggctgtaggcataaaa

SEQ ID NO: 17 - RNA, 21 nt, synthetic construct
  source 1..21: mol_type = other RNA
aggctgtaggcataaattgga

SEQ ID NO: 18 - RNA, 21 nt, synthetic construct
  source 1..21: mol_type = other RNA
cttctctcaattttctaggga

SEQ ID NO: 19 - RNA, 21 nt, synthetic construct
  source 1..21: mol_type = other RNA
ctgttaccaattttcttttga

SEQ ID NO: 20 - RNA, 21 nt, synthetic construct
  source 1..21: mol_type = other RNA
ccgtctgtgccttctcatcta

SEQ ID NO: 21 - RNA, 21 nt, synthetic construct
  source 1..21: mol_type = other RNA
tacataagaggactcttggaa

SEQ ID NO: 22 - RNA, 21 nt, synthetic construct
  source 1..21: mol_type = other RNA
tacaggcggggtttttcttga

SEQ ID NO: 23 - RNA, 21 nt, synthetic construct
  source 1..21: mol_type = other RNA
caggcggggtttttcttgtta

SEQ ID NO: 24 - RNA, 21 nt, synthetic construct
  source 1..21: mol_type = other RNA
cggggtttttcttgttgacaa

SEQ ID NO: 25 - RNA, 21 nt, synthetic construct
  source 1..21: mol_type = other RNA
ctcgtggtggacttctctcaa

SEQ ID NO: 26 - RNA, 21 nt, synthetic construct
  source 1..21: mol_type = other RNA
cgtggtggacttctctcaata

SEQ ID NO: 27 - RNA, 21 nt, synthetic construct
  source 1..21: mol_type = other RNA
gtggtggacttctctcaatta

SEQ ID NO: 28 - RNA, 21 nt, synthetic construct
  source 1..21: mol_type = other RNA
tttactagtgccatttgttca

SEQ ID NO: 29 - RNA, 21 nt, synthetic construct
  source 1..21: mol_type = other RNA
agtgccatttgttcagtggta

SEQ ID NO: 30 - RNA, 21 nt, synthetic construct
  source 1..21: mol_type = other RNA
ttaccaattttcttttgtcta

SEQ ID NO: 31 - RNA, 21 nt, synthetic construct
  source 1..21: mol_type = other RNA
aggcctattgattggaaagta

SEQ ID NO: 32 - RNA, 21 nt, synthetic construct
  source 1..21: mol_type = other RNA
ccgatccatactgcggaacta

SEQ ID NO: 33 - RNA, 21 nt, synthetic construct
  source 1..21: mol_type = other RNA
gtgtgcacttcgcttcaccta

SEQ ID NO: 34 - RNA, 21 nt, synthetic construct
  source 1..21: mol_type = other RNA
ttacataagaggactcttgga

SEQ ID NO: 35 - RNA, 21 nt, synthetic construct
  source 1..21: mol_type = other RNA
tcctgctgctatgcctcatca

SEQ ID NO: 36 - RNA, 21 nt, synthetic construct
  source 1..21: mol_type = other RNA
ctgtgccaagtgtttgctgaa

SEQ ID NO: 37 - RNA, 21 nt, synthetic construct
  source 1..21: mol_type = other RNA
tgtgccaagtgtttgctgaca

SEQ ID NO: 38 - RNA, 21 nt, synthetic construct
  source 1..21: mol_type = other RNA
cgtgtgcacttcgcttcacca

SEQ ID NO: 39 - RNA, 21 nt, synthetic construct
  source 1..21: mol_type = other RNA
gtataagaggactcttggaca

SEQ ID NO: 40 - RNA, 21 nt, synthetic construct
  source 1..21: mol_type = other RNA
gtctagactcgtggtggacta

SEQ ID NO: 41 - RNA, 21 nt, synthetic construct
  source 1..21: mol_type = other RNA
tctagactcgtggtggactta

SEQ ID NO: 42 - RNA, 21 nt, synthetic construct
  source 1..21: mol_type = other RNA
atcctgctgctatgcctcata

SEQ ID NO: 43 - RNA, 21 nt, synthetic construct
  source 1..21: mol_type = other RNA
aaggtatgttgcccgtttgta

SEQ ID NO: 44 - RNA, 21 nt, synthetic construct
  source 1..21: mol_type = other RNA
agtttactagtgccatttgta

SEQ ID NO: 45 - RNA, 21 nt, synthetic construct
  source 1..21: mol_type = other RNA
ccatttgttcagtggttcgta

SEQ ID NO: 46 - RNA, 21 nt, synthetic construct
  source 1..21: mol_type = other RNA
cagcgcatgcgtggaacctta

SEQ ID NO: 47 - RNA, 21 nt, synthetic construct
  source 1..21: mol_type = other RNA
atgtcaacgaccgaccttgaa

SEQ ID NO: 48 - RNA, 21 nt, synthetic construct
  source 1..21: mol_type = other RNA
gttacaggcggggtttttcta

SEQ ID NO: 49 - RNA, 21 nt, synthetic construct
  source 1..21: mol_type = other RNA
gcagagtctagactcgtggta

SEQ ID NO: 50 - RNA, 21 nt, synthetic construct
  source 1..21: mol_type = other RNA
gagtctagactcgtggtggaa

SEQ ID NO: 51 - RNA, 21 nt, synthetic construct
  source 1..21: mol_type = other RNA
cttcatcctgctgctatgcca

SEQ ID NO: 52 - RNA, 21 nt, synthetic construct
  source 1..21: mol_type = other RNA
cctgctgctatgcctcatcta

SEQ ID NO: 53 - RNA, 21 nt, synthetic construct
  source 1..21: mol_type = other RNA
aggtatgttgcccgtttgtca

SEQ ID NO: 54 - RNA, 21 nt, synthetic construct
  source 1..21: mol_type = other RNA
gtgccatttgttcagtggtta

SEQ ID NO: 55 - RNA, 21 nt, synthetic construct
  source 1..21: mol_type = other RNA
cggggcgcacctctctttaca

SEQ ID NO: 56 - RNA, 21 nt, synthetic construct
  source 1..21: mol_type = other RNA
ttacaggcggggtttttctta

SEQ ID NO: 57 - RNA, 21 nt, synthetic construct
  source 1..21: mol_type = other RNA
acaggcggggtttttcttgta

SEQ ID NO: 58 - RNA, 21 nt, synthetic construct
  source 1..21: mol_type = other RNA
tcaaggtatgttgcccgttta

SEQ ID NO: 59 - RNA, 21 nt, synthetic construct
  source 1..21: mol_type = other RNA
catactgcggaactcctagca

SEQ ID NO: 60 - RNA, 21 nt, synthetic construct
  source 1..21: mol_type = other RNA
gaccacggggcgcacctctca

SEQ ID NO: 61 - RNA, 21 nt, synthetic construct
  source 1..21: mol_type = other RNA
tgtcaacgaccgaccttgaga

SEQ ID NO: 62 - RNA, 21 nt, synthetic construct
  source 1..21: mol_type = other RNA
ttcatcctgctgctatgccta

SEQ ID NO: 63 - RNA, 21 nt, synthetic construct
  source 1..21: mol_type = other RNA
gctcctctgccgatccataca

SEQ ID NO: 64 - RNA, 21 nt, synthetic construct
  source 1..21: mol_type = other RNA
ctcctctgccgatccatacta

SEQ ID NO: 65 - RNA, 21 nt, synthetic construct
  source 1..21: mol_type = other RNA
cctctgccgatccatactgca

SEQ ID NO: 66 - RNA, 21 nt, synthetic construct
  source 1..21: mol_type = other RNA
cgatccatactgcggaactca

SEQ ID NO: 67 - RNA, 21 nt, synthetic construct
  source 1..21: mol_type = other RNA
ggcgcacctctctttacgcga

SEQ ID NO: 68 - RNA, 21 nt, synthetic construct
  source 1..21: mol_type = other RNA
cccgtctgtgccttctcatca

SEQ ID NO: 69 - RNA, 21 nt, synthetic construct
  source 1..21: mol_type = other RNA
tcaacgaccgaccttgaggca

SEQ ID NO: 70 - RNA, 19 nt, synthetic construct
  source 1..19: mol_type = other RNA
gtggacttctctcaattta

SEQ ID NO: 71 - RNA, 19 nt, synthetic construct
  source 1..19: mol_type = other RNA
ttctctcaattttctagga

SEQ ID NO: 72 - RNA, 19 nt, synthetic construct
  source 1..19: mol_type = other RNA
taccaattttcttttgtca

SEQ ID NO: 73 - RNA, 19 nt, synthetic construct
  source 1..19: mol_type = other RNA
taagaggactcttggacta

SEQ ID NO: 74 - RNA, 19 nt, synthetic construct
  source 1..19: mol_type = other RNA
ggtttttcttgttgacaaa

SEQ ID NO: 75 - RNA, 19 nt, synthetic construct
  source 1..19: mol_type = other RNA
gacttctctcaattttcta

SEQ ID NO: 76 - RNA, 19 nt, synthetic construct
  source 1..19: mol_type = other RNA
gctatgcctcatcttctta

SEQ ID NO: 77 - RNA, 19 nt, synthetic construct
  source 1..19: mol_type = other RNA
tttgttcagtggttcgtaa

SEQ ID NO: 78 - RNA, 19 nt, synthetic construct
  source 1..19: mol_type = other RNA
gcgcacctctctttacgca

SEQ ID NO: 79 - RNA, 19 nt, synthetic construct
  source 1..19: mol_type = other RNA
gactcgtggtggacttcta

SEQ ID NO: 80 - RNA, 19 nt, synthetic construct
  source 1..19: mol_type = other RNA
acttctctcaattttctaa

SEQ ID NO: 81 - RNA, 19 nt, synthetic construct
  source 1..19: mol_type = other RNA
ggctcagtttactagtgca

SEQ ID NO: 82 - RNA, 19 nt, synthetic construct
  source 1..19: mol_type = other RNA
agtgccatttgttcagtga

SEQ ID NO: 83 - RNA, 19 nt, synthetic construct
  source 1..19: mol_type = other RNA
ttaccaattttcttttgta

SEQ ID NO: 84 - RNA, 19 nt, synthetic construct
  source 1..19: mol_type = other RNA
cgcttcacctctgcacgta

SEQ ID NO: 85 - RNA, 19 nt, synthetic construct
  source 1..19: mol_type = other RNA
ggaggctgtaggcataaaa

SEQ ID NO: 86 - RNA, 19 nt, synthetic construct
  source 1..19: mol_type = other RNA
gctgtaggcataaattgga

SEQ ID NO: 87 - RNA, 19 nt, synthetic construct
  source 1..19: mol_type = other RNA
tctctcaattttctaggga

SEQ ID NO: 88 - RNA, 19 nt, synthetic construct
  source 1..19: mol_type = other RNA
gttaccaattttcttttga

SEQ ID NO: 89 - RNA, 19 nt, synthetic construct
  source 1..19: mol_type = other RNA
gtctgtgccttctcatcta

SEQ ID NO: 90 - RNA, 19 nt, synthetic construct
  source 1..19: mol_type = other RNA
cataagaggactcttggaa

SEQ ID NO: 91 - RNA, 19 nt, synthetic construct
  source 1..19: mol_type = other RNA
caggcggggtttttcttga

SEQ ID NO: 92 - RNA, 19 nt, synthetic construct
  source 1..19: mol_type = other RNA
ggcggggtttttcttgtta

SEQ ID NO: 93 - RNA, 19 nt, synthetic construct
  source 1..19: mol_type = other RNA
gggtttttcttgttgacaa

SEQ ID NO: 94 - RNA, 19 nt, synthetic construct
  source 1..19: mol_type = other RNA
cgtggtggacttctctcaa

SEQ ID NO: 95 - RNA, 19 nt, synthetic construct
  source 1..19: mol_type = other RNA
tggtggacttctctcaata

SEQ ID NO: 96 - RNA, 19 nt, synthetic construct
  source 1..19: mol_type = other RNA
ggtggacttctctcaatta

SEQ ID NO: 97 - RNA, 19 nt, synthetic construct
  source 1..19: mol_type = other RNA
tactagtgccatttgttca

SEQ ID NO: 98 - RNA, 19 nt, synthetic construct
  source 1..19: mol_type = other RNA
tgccatttgttcagtggta

SEQ ID NO: 99 - RNA, 19 nt, synthetic construct
  source 1..19: mol_type = other RNA
accaattttcttttgtcta

SEQ ID NO: 100 - RNA, 19 nt, synthetic construct
  source 1..19: mol_type = other RNA
gcctattgattggaaagta

SEQ ID NO: 101 - RNA, 19 nt, synthetic construct
  source 1..19: mol_type = other RNA
gatccatactgcggaacta

SEQ ID NO: 102 - RNA, 19 nt, synthetic construct
  source 1..19: mol_type = other RNA
gtgcacttcgcttcaccta

SEQ ID NO: 103 - RNA, 19 nt, synthetic construct
  source 1..19: mol_type = other RNA
acataagaggactcttgga

SEQ ID NO: 104 - RNA, 19 nt, synthetic construct
  source 1..19: mol_type = other RNA
ctgctgctatgcctcatca

SEQ ID NO: 105 - RNA, 19 nt, synthetic construct
  source 1..19: mol_type = other RNA
gtgccaagtgtttgctgaa

SEQ ID NO: 106 - RNA, 19 nt, synthetic construct
  source 1..19: mol_type = other RNA
tgccaagtgtttgctgaca

SEQ ID NO: 107 - RNA, 19 nt, synthetic construct
  source 1..19: mol_type = other RNA
tgtgcacttcgcttcacca

SEQ ID NO: 108 - RNA, 19 nt, synthetic construct
  source 1..19: mol_type = other RNA
ataagaggactcttggaca

SEQ ID NO: 109 - RNA, 19 nt, synthetic construct
  source 1..19: mol_type = other RNA
ctagactcgtggtggacta

SEQ ID NO: 110 - RNA, 19 nt, synthetic construct
  source 1..19: mol_type = other RNA
tagactcgtggtggactta

SEQ ID NO: 111 - RNA, 19 nt, synthetic construct
  source 1..19: mol_type = other RNA
cctgctgctatgcctcata

SEQ ID NO: 112 - RNA, 19 nt, synthetic construct
  source 1..19: mol_type = other RNA
ggtatgttgcccgtttgta

SEQ ID NO: 113 - RNA, 19 nt, synthetic construct
  source 1..19: mol_type = other RNA
tttactagtgccatttgta

SEQ ID NO: 114 - RNA, 19 nt, synthetic construct
  source 1..19: mol_type = other RNA
atttgttcagtggttcgta

SEQ ID NO: 115 - RNA, 19 nt, synthetic construct
  source 1..19: mol_type = other RNA
gcgcatgcgtggaacctta

SEQ ID NO: 116 - RNA, 19 nt, synthetic construct
  source 1..19: mol_type = other RNA
gtcaacgaccgaccttgaa

SEQ ID NO: 117 - RNA, 19 nt, synthetic construct
  source 1..19: mol_type = other RNA
tacaggcggggtttttcta

SEQ ID NO: 118 - RNA, 19 nt, synthetic construct
  source 1..19: mol_type = other RNA
agagtctagactcgtggta

SEQ ID NO: 119 - RNA, 19 nt, synthetic construct
  source 1..19: mol_type = other RNA
gtctagactcgtggtggaa

SEQ ID NO: 120 - RNA, 19 nt, synthetic construct
  source 1..19: mol_type = other RNA
tcatcctgctgctatgcca

SEQ ID NO: 121 - RNA, 19 nt, synthetic construct
  source 1..19: mol_type = other RNA
tgctgctatgcctcatcta

SEQ ID NO: 122 - RNA, 19 nt, synthetic construct
  source 1..19: mol_type = other RNA
gtatgttgcccgtttgtca

SEQ ID NO: 123 - RNA, 19 nt, synthetic construct
  source 1..19: mol_type = other RNA
gccatttgttcagtggtta

SEQ ID NO: 124 - RNA, 19 nt, synthetic construct
  source 1..19: mol_type = other RNA
gggcgcacctctctttaca

SEQ ID NO: 125 - RNA, 19 nt, synthetic construct
  source 1..19: mol_type = other RNA
acaggcggggtttttctta

SEQ ID NO: 126 - RNA, 19 nt, synthetic construct
  source 1..19: mol_type = other RNA
aggcggggtttttcttgta

SEQ ID NO: 127 - RNA, 19 nt, synthetic construct
  source 1..19: mol_type = other RNA
aaggtatgttgcccgttta

SEQ ID NO: 128 - RNA, 19 nt, synthetic construct
  source 1..19: mol_type = other RNA
tactgcggaactcctagca

SEQ ID NO: 129 - RNA, 19 nt, synthetic construct
  source 1..19: mol_type = other RNA
ccacggggcgcacctctca

SEQ ID NO: 130 - RNA, 19 nt, synthetic construct
  source 1..19: mol_type = other RNA
tcaacgaccgaccttgaga

SEQ ID NO: 131 - RNA, 19 nt, synthetic construct
  source 1..19: mol_type = other RNA
catcctgctgctatgccta

SEQ ID NO: 132 - RNA, 19 nt, synthetic construct
  source 1..19: mol_type = other RNA
tcctctgccgatccataca

SEQ ID NO: 133 - RNA, 19 nt, synthetic construct
  source 1..19: mol_type = other RNA
cctctgccgatccatacta

SEQ ID NO: 134 - RNA, 19 nt, synthetic construct
  source 1..19: mol_type = other RNA
tctgccgatccatactgca

SEQ ID NO: 135 - RNA, 19 nt, synthetic construct
  source 1..19: mol_type = other RNA
atccatactgcggaactca

SEQ ID NO: 136 - RNA, 19 nt, synthetic construct
  source 1..19: mol_type = other RNA
cgcacctctctttacgcga

SEQ ID NO: 137 - RNA, 19 nt, synthetic construct
  source 1..19: mol_type = other RNA
cgtctgtgccttctcatca

SEQ ID NO: 138 - RNA, 19 nt, synthetic construct
  source 1..19: mol_type = other RNA
aacgaccgaccttgaggca

SEQ ID NO: 139 - RNA, 21 nt, synthetic construct
  source 1..21: mol_type = other RNA
taaattgagagaagtccacca

SEQ ID NO: 140 - RNA, 21 nt, synthetic construct
  source 1..21: mol_type = other RNA
tcctagaaaattgagagaagt

SEQ ID NO: 141 - RNA, 21 nt, synthetic construct
  source 1..21: mol_type = other RNA
tgacaaaagaaaattggtaac

SEQ ID NO: 142 - RNA, 21 nt, synthetic construct
  source 1..21: mol_type = other RNA
tagtccaagagtcctcttatg

SEQ ID NO: 143 - RNA, 21 nt, synthetic construct
  source 1..21: mol_type = other RNA
tttgtcaacaagaaaaacccc

SEQ ID NO: 144 - RNA, 21 nt, synthetic construct
  source 1..21: mol_type = other RNA
tagaaaattgagagaagtcca

SEQ ID NO: 145 - RNA, 21 nt, synthetic construct
  source 1..21: mol_type = other RNA
taagaagatgaggcatagcag

SEQ ID NO: 146 - RNA, 21 nt, synthetic construct
  source 1..21: mol_type = other RNA
ttacgaaccactgaacaaatg

SEQ ID NO: 147 - RNA, 21 nt, synthetic construct
  source 1..21: mol_type = other RNA
tgcgtaaagagaggtgcgccc

SEQ ID NO: 148 - RNA, 21 nt, synthetic construct
  source 1..21: mol_type = other RNA
tagaagtccaccacgagtcta

SEQ ID NO: 149 - RNA, 21 nt, synthetic construct
  source 1..21: mol_type = other RNA
ttagaaaattgagagaagtcc

SEQ ID NO: 150 - RNA, 21 nt, synthetic construct
  source 1..21: mol_type = other RNA
tgcactagtaaactgagccaa

SEQ ID NO: 151 - RNA, 21 nt, synthetic construct
  source 1..21: mol_type = other RNA
tcactgaacaaatggcactag

SEQ ID NO: 152 - RNA, 21 nt, synthetic construct
  source 1..21: mol_type = other RNA
tacaaaagaaaattggtaaca

SEQ ID NO: 153 - RNA, 21 nt, synthetic construct
  source 1..21: mol_type = other RNA
tacgtgcagaggtgaagcgaa

SEQ ID NO: 154 - RNA, 21 nt, synthetic construct
  source 1..21: mol_type = other RNA
ttttatgcctacagcctccta

SEQ ID NO: 155 - RNA, 21 nt, synthetic construct
  source 1..21: mol_type = other RNA
tccaatttatgcctacagcct

SEQ ID NO: 156 - RNA, 21 nt, synthetic construct
  source 1..21: mol_type = other RNA
tccctagaaaattgagagaag

SEQ ID NO: 157 - RNA, 21 nt, synthetic construct
  source 1..21: mol_type = other RNA
tcaaaagaaaattggtaacag

SEQ ID NO: 158 - RNA, 21 nt, synthetic construct
  source 1..21: mol_type = other RNA
tagatgagaaggcacagacgg

SEQ ID NO: 159 - RNA, 21 nt, synthetic construct
  source 1..21: mol_type = other RNA
ttccaagagtcctcttatgta

SEQ ID NO: 160 - RNA, 21 nt, synthetic construct
  source 1..21: mol_type = other RNA
tcaagaaaaaccccgcctgta

SEQ ID NO: 161 - RNA, 21 nt, synthetic construct
  source 1..21: mol_type = other RNA
taacaagaaaaaccccgcctg

SEQ ID NO: 162 - RNA, 21 nt, synthetic construct
  source 1..21: mol_type = other RNA
ttgtcaacaagaaaaaccccg

SEQ ID NO: 163 - RNA, 21 nt, synthetic construct
  source 1..21: mol_type = other RNA
ttgagagaagtccaccacgag

SEQ ID NO: 164 - RNA, 21 nt, synthetic construct
  source 1..21: mol_type = other RNA
tattgagagaagtccaccacg

SEQ ID NO: 165 - RNA, 21 nt, synthetic construct
  source 1..21: mol_type = other RNA
taattgagagaagtccaccac

SEQ ID NO: 166 - RNA, 21 nt, synthetic construct
  source 1..21: mol_type = other RNA
tgaacaaatggcactagtaaa

SEQ ID NO: 167 - RNA, 21 nt, synthetic construct
  source 1..21: mol_type = other RNA
taccactgaacaaatggcact

SEQ ID NO: 168 - RNA, 21 nt, synthetic construct
  source 1..21: mol_type = other RNA
tagacaaaagaaaattggtaa

SEQ ID NO: 169 - RNA, 21 nt, synthetic construct
  source 1..21: mol_type = other RNA
tactttccaatcaataggcct

SEQ ID NO: 170 - RNA, 21 nt, synthetic construct
  source 1..21: mol_type = other RNA
tagttccgcagtatggatcgg

SEQ ID NO: 171 - RNA, 21 nt, synthetic construct
  source 1..21: mol_type = other RNA
taggtgaagcgaagtgcacac

SEQ ID NO: 172 - RNA, 21 nt, synthetic construct
  source 1..21: mol_type = other RNA
tccaagagtcctcttatgtaa

SEQ ID NO: 173 - RNA, 21 nt, synthetic construct
  source 1..21: mol_type = other RNA
tgatgaggcatagcagcagga

SEQ ID NO: 174 - RNA, 21 nt, synthetic construct
  source 1..21: mol_type = other RNA
ttcagcaaacacttggcacag

SEQ ID NO: 175 - RNA, 21 nt, synthetic construct
  source 1..21: mol_type = other RNA
tgtcagcaaacacttggcaca

SEQ ID NO: 176 - RNA, 21 nt, synthetic construct
  source 1..21: mol_type = other RNA
tggtgaagcgaagtgcacacg

SEQ ID NO: 177 - RNA, 21 nt, synthetic construct
  source 1..21: mol_type = other RNA
tgtccaagagtcctcttatac

SEQ ID NO: 178 - RNA, 21 nt, synthetic construct
  source 1..21: mol_type = other RNA
tagtccaccacgagtctagac

SEQ ID NO: 179 - RNA, 21 nt, synthetic construct
  source 1..21: mol_type = other RNA
taagtccaccacgagtctaga

SEQ ID NO: 180 - RNA, 21 nt, synthetic construct
  source 1..21: mol_type = other RNA
tatgaggcatagcagcaggat

SEQ ID NO: 181 - RNA, 21 nt, synthetic construct
  source 1..21: mol_type = other RNA
tacaaacgggcaacatacctt

SEQ ID NO: 182 - RNA, 21 nt, synthetic construct
  source 1..21: mol_type = other RNA
tacaaatggcactagtaaact

SEQ ID NO: 183 - RNA, 21 nt, synthetic construct
  source 1..21: mol_type = other RNA
tacgaaccactgaacaaatgg

SEQ ID NO: 184 - RNA, 21 nt, synthetic construct
  source 1..21: mol_type = other RNA
taaggttccacgcatgcgctg

SEQ ID NO: 185 - RNA, 21 nt, synthetic construct
  source 1..21: mol_type = other RNA
ttcaaggtcggtcgttgacat

SEQ ID NO: 186 - RNA, 21 nt, synthetic construct
  source 1..21: mol_type = other RNA
tagaaaaaccccgcctgtaac

SEQ ID NO: 187 - RNA, 21 nt, synthetic construct
  source 1..21: mol_type = other RNA
taccacgagtctagactctgc

SEQ ID NO: 188 - RNA, 21 nt, synthetic construct
  source 1..21: mol_type = other RNA
ttccaccacgagtctagactc

SEQ ID NO: 189 - RNA, 21 nt, synthetic construct
  source 1..21: mol_type = other RNA
tggcatagcagcaggatgaag

SEQ ID NO: 190 - RNA, 21 nt, synthetic construct
  source 1..21: mol_type = other RNA
tagatgaggcatagcagcagg

SEQ ID NO: 191 - RNA, 21 nt, synthetic construct
  source 1..21: mol_type = other RNA
tgacaaacgggcaacatacct

SEQ ID NO: 192 - RNA, 21 nt, synthetic construct
  source 1..21: mol_type = other RNA
taaccactgaacaaatggcac

SEQ ID NO: 193 - RNA, 21 nt, synthetic construct
  source 1..21: mol_type = other RNA
tgtaaagagaggtgcgccccg

SEQ ID NO: 194 - RNA, 21 nt, synthetic construct
  source 1..21: mol_type = other RNA
taagaaaaaccccgcctgtaa

SEQ ID NO: 195 - RNA, 21 nt, synthetic construct
  source 1..21: mol_type = other RNA
tacaagaaaaaccccgcctgt

SEQ ID NO: 196 - RNA, 21 nt, synthetic construct
  source 1..21: mol_type = other RNA
taaacgggcaacataccttga

SEQ ID NO: 197 - RNA, 21 nt, synthetic construct
  source 1..21: mol_type = other RNA
tgctaggagttccgcagtatg

SEQ ID NO: 198 - RNA, 21 nt, synthetic construct
  source 1..21: mol_type = other RNA
tgagaggtgcgccccgtggtc

SEQ ID NO: 199 - RNA, 21 nt, synthetic construct
  source 1..21: mol_type = other RNA
tctcaaggtcggtcgttgaca

SEQ ID NO: 200 - RNA, 21 nt, synthetic construct
  source 1..21: mol_type = other RNA
taggcatagcagcaggatgaa

SEQ ID NO: 201 - RNA, 21 nt, synthetic construct
  source 1..21: mol_type = other RNA
tgtatggatcggcagaggagc

SEQ ID NO: 202 - RNA, 21 nt, synthetic construct
  source 1..21: mol_type = other RNA
tagtatggatcggcagaggag

SEQ ID NO: 203 - RNA, 21 nt, synthetic construct
  source 1..21: mol_type = other RNA
tgcagtatggatcggcagagg

SEQ ID NO: 204 - RNA, 21 nt, synthetic construct
  source 1..21: mol_type = other RNA
tgagttccgcagtatggatcg

SEQ ID NO: 205 - RNA, 21 nt, synthetic construct
  source 1..21: mol_type = other RNA
tcgcgtaaagagaggtgcgcc

SEQ ID NO: 206 - RNA, 21 nt, synthetic construct
  source 1..21: mol_type = other RNA
tgatgagaaggcacagacggg

SEQ ID NO: 207 - RNA, 21 nt, synthetic construct
  source 1..21: mol_type = other RNA
tgcctcaaggtcggtcgttga

SEQ ID NO: 208 - RNA, 19 nt, synthetic construct
  source 1..19: mol_type = other RNA
taaattgagagaagtccac

SEQ ID NO: 209 - RNA, 19 nt, synthetic construct
  source 1..19: mol_type = other RNA
tcctagaaaattgagagaa

SEQ ID NO: 210 - RNA, 19 nt, synthetic construct
  source 1..19: mol_type = other RNA
tgacaaaagaaaattggta

SEQ ID NO: 211 - RNA, 19 nt, synthetic construct
  source 1..19: mol_type = other RNA
tagtccaagagtcctctta

SEQ ID NO: 212 - RNA, 19 nt, synthetic construct
  source 1..19: mol_type = other RNA
tttgtcaacaagaaaaacc

SEQ ID NO: 213 - RNA, 19 nt, synthetic construct
  source 1..19: mol_type = other RNA
tagaaaattgagagaagtc

SEQ ID NO: 214 - RNA, 19 nt, synthetic construct
  source 1..19: mol_type = other RNA
taagaagatgaggcatagc

SEQ ID NO: 215 - RNA, 19 nt, synthetic construct
  source 1..19: mol_type = other RNA
ttacgaaccactgaacaaa

SEQ ID NO: 216 - RNA, 19 nt, synthetic construct
  source 1..19: mol_type = other RNA
tgcgtaaagagaggtgcgc

SEQ ID NO: 217 - RNA, 19 nt, synthetic construct
  source 1..19: mol_type = other RNA
tagaagtccaccacgagtc

SEQ ID NO: 218 - RNA, 19 nt, synthetic construct
  source 1..19: mol_type = other RNA
ttagaaaattgagagaagt

SEQ ID NO: 219 - RNA, 19 nt, synthetic construct
  source 1..19: mol_type = other RNA
tgcactagtaaactgagcc

SEQ ID NO: 220 - RNA, 19 nt, synthetic construct
  source 1..19: mol_type = other RNA
tcactgaacaaatggcact

SEQ ID NO: 221 - RNA, 19 nt, synthetic construct
  source 1..19: mol_type = other RNA
tacaaaagaaaattggtaa

SEQ ID NO: 222 - RNA, 19 nt, synthetic construct
  source 1..19: mol_type = other RNA
tacgtgcagaggtgaagcg

SEQ ID NO: 223 - RNA, 19 nt, synthetic construct
  source 1..19: mol_type = other RNA
ttttatgcctacagcctcc

SEQ ID NO: 224 - RNA, 19 nt, synthetic construct
  source 1..19: mol_type = other RNA
tccaatttatgcctacagc

SEQ ID NO: 225 - RNA, 19 nt, synthetic construct
  source 1..19: mol_type = other RNA
tccctagaaaattgagaga

SEQ ID NO: 226 - RNA, 19 nt, synthetic construct
  source 1..19: mol_type = other RNA
tcaaaagaaaattggtaac

SEQ ID NO: 227 - RNA, 19 nt, synthetic construct
  source 1..19: mol_type = other RNA
tagatgagaaggcacagac

SEQ ID NO: 228 - RNA, 19 nt, synthetic construct
  source 1..19: mol_type = other RNA
ttccaagagtcctcttatg

SEQ ID NO: 229 - RNA, 19 nt, synthetic construct
  source 1..19: mol_type = other RNA
tcaagaaaaaccccgcctg

SEQ ID NO: 230 - RNA, 19 nt, synthetic construct
  source 1..19: mol_type = other RNA
taacaagaaaaaccccgcc

SEQ ID NO: 231 - RNA, 19 nt, synthetic construct
  source 1..19: mol_type = other RNA
ttgtcaacaagaaaaaccc

SEQ ID NO: 232 - RNA, 19 nt, synthetic construct
  source 1..19: mol_type = other RNA
ttgagagaagtccaccacg

SEQ ID NO: 233 - RNA, 19 nt, synthetic construct
  source 1..19: mol_type = other RNA
tattgagagaagtccacca

SEQ ID NO: 234 - RNA, 19 nt, synthetic construct
  source 1..19: mol_type = other RNA
taattgagagaagtccacc

SEQ ID NO: 235 - RNA, 19 nt, synthetic construct
  source 1..19: mol_type = other RNA
tgaacaaatggcactagta

SEQ ID NO: 236 - RNA, 19 nt, synthetic construct
  source 1..19: mol_type = other RNA
taccactgaacaaatggca

SEQ ID NO: 237 - RNA, 19 nt, synthetic construct
  source 1..19: mol_type = other RNA
tagacaaaagaaaattggt

SEQ ID NO: 238 - RNA, 19 nt, synthetic construct
  source 1..19: mol_type = other RNA
tactttccaatcaataggc

SEQ ID NO: 239 - RNA, 19 nt, synthetic construct
  source 1..19: mol_type = other RNA
tagttccgcagtatggatc

SEQ ID NO: 240 - RNA, 19 nt, synthetic construct
  source 1..19: mol_type = other RNA
taggtgaagcgaagtgcac

SEQ ID NO: 241 - RNA, 19 nt, synthetic construct
  source 1..19: mol_type = other RNA
tccaagagtcctcttatgt

SEQ ID NO: 242 - RNA, 19 nt, synthetic construct
  source 1..19: mol_type = other RNA
tgatgaggcatagcagcag

SEQ ID NO: 243 - RNA, 19 nt, synthetic construct
  source 1..19: mol_type = other RNA
ttcagcaaacacttggcac

SEQ ID NO: 244 - RNA, 19 nt, synthetic construct
  source 1..19: mol_type = other RNA
tgtcagcaaacacttggca

SEQ ID NO: 245 - RNA, 19 nt, synthetic construct
  source 1..19: mol_type = other RNA
tggtgaagcgaagtgcaca

SEQ ID NO: 246 - RNA, 19 nt, synthetic construct
  source 1..19: mol_type = other RNA
tgtccaagagtcctcttat

SEQ ID NO: 247 - RNA, 19 nt, synthetic construct
  source 1..19: mol_type = other RNA
tagtccaccacgagtctag

SEQ ID NO: 248 - RNA, 19 nt, synthetic construct
  source 1..19: mol_type = other RNA
taagtccaccacgagtcta

SEQ ID NO: 249 - RNA, 19 nt, synthetic construct
  source 1..19: mol_type = other RNA
tatgaggcatagcagcagg

SEQ ID NO: 250 - RNA, 19 nt, synthetic construct
  source 1..19: mol_type = other RNA
tacaaacgggcaacatacc

SEQ ID NO: 251 - RNA, 19 nt, synthetic construct
  source 1..19: mol_type = other RNA
tacaaatggcactagtaaa

SEQ ID NO: 252 - RNA, 19 nt, synthetic construct
  source 1..19: mol_type = other RNA
tacgaaccactgaacaaat

SEQ ID NO: 253 - RNA, 19 nt, synthetic construct
  source 1..19: mol_type = other RNA
taaggttccacgcatgcgc

SEQ ID NO: 254 - RNA, 19 nt, synthetic construct
  source 1..19: mol_type = other RNA
ttcaaggtcggtcgttgac

SEQ ID NO: 255 - RNA, 19 nt, synthetic construct
  source 1..19: mol_type = other RNA
tagaaaaaccccgcctgta

SEQ ID NO: 256 - RNA, 19 nt, synthetic construct
  source 1..19: mol_type = other RNA
taccacgagtctagactct

SEQ ID NO: 257 - RNA, 19 nt, synthetic construct
  source 1..19: mol_type = other RNA
ttccaccacgagtctagac

SEQ ID NO: 258 - RNA, 19 nt, synthetic construct
  source 1..19: mol_type = other RNA
tggcatagcagcaggatga

SEQ ID NO: 259 - RNA, 19 nt, synthetic construct
  source 1..19: mol_type = other RNA
tagatgaggcatagcagca

SEQ ID NO: 260 - RNA, 19 nt, synthetic construct
  source 1..19: mol_type = other RNA
tgacaaacgggcaacatac

SEQ ID NO: 261 - RNA, 19 nt, synthetic construct
  source 1..19: mol_type = other RNA
taaccactgaacaaatggc

SEQ ID NO: 262 - RNA, 19 nt, synthetic construct
  source 1..19: mol_type = other RNA
tgtaaagagaggtgcgccc

SEQ ID NO: 263 - RNA, 19 nt, synthetic construct
  source 1..19: mol_type = other RNA
taagaaaaaccccgcctgt

SEQ ID NO: 264 - RNA, 19 nt, synthetic construct
  source 1..19: mol_type = other RNA
tacaagaaaaaccccgcct

SEQ ID NO: 265 - RNA, 19 nt, synthetic construct
  source 1..19: mol_type = other RNA
taaacgggcaacatacctt

SEQ ID NO: 266 - RNA, 19 nt, synthetic construct
  source 1..19: mol_type = other RNA
tgctaggagttccgcagta

SEQ ID NO: 267 - RNA, 19 nt, synthetic construct
  source 1..19: mol_type = other RNA
tgagaggtgcgccccgtgg

SEQ ID NO: 268 - RNA, 19 nt, synthetic construct
  source 1..19: mol_type = other RNA
tctcaaggtcggtcgttga

SEQ ID NO: 269 - RNA, 19 nt, synthetic construct
  source 1..19: mol_type = other RNA
taggcatagcagcaggatg

SEQ ID NO: 270 - RNA, 19 nt, synthetic construct
  source 1..19: mol_type = other RNA
tgtatggatcggcagagga

SEQ ID NO: 271 - RNA, 19 nt, synthetic construct
  source 1..19: mol_type = other RNA
tagtatggatcggcagagg

SEQ ID NO: 272 - RNA, 19 nt, synthetic construct
  source 1..19: mol_type = other RNA
tgcagtatggatcggcaga

SEQ ID NO: 273 - RNA, 19 nt, synthetic construct
  source 1..19: mol_type = other RNA
tgagttccgcagtatggat

SEQ ID NO: 274 - RNA, 19 nt, synthetic construct
  source 1..19: mol_type = other RNA
tcgcgtaaagagaggtgcg

SEQ ID NO: 275 - RNA, 19 nt, synthetic construct
  source 1..19: mol_type = other RNA
tgatgagaaggcacagacg

SEQ ID NO: 276 - RNA, 19 nt, synthetic construct
  source 1..19: mol_type = other RNA
tgcctcaaggtcggtcgtt

SEQ ID NO: 277 - RNA, 21 nt, synthetic construct
  source 1..21: mol_type = other RNA
tggtggacttctctcaattta

SEQ ID NO: 278 - RNA, 21 nt, synthetic construct
  source 1..21: mol_type = other RNA
acttctctcaattttctagga

SEQ ID NO: 279 - RNA, 21 nt, synthetic construct
  source 1..21: mol_type = other RNA
gttaccaattttcttttgtca

SEQ ID NO: 280 - RNA, 21 nt, synthetic construct
  source 1..21: mol_type = other RNA
cataagaggactcttggacta

SEQ ID NO: 281 - RNA, 21 nt, synthetic construct
  source 1..21: mol_type = other RNA
ggggtttttcttgttgacaaa

SEQ ID NO: 282 - RNA, 21 nt, synthetic construct
  source 1..21: mol_type = other RNA
tggacttctctcaattttcta

SEQ ID NO: 283 - RNA, 21 nt, synthetic construct
  source 1..21: mol_type = other RNA
ctgctatgcctcatcttctta

SEQ ID NO: 284 - RNA, 21 nt, synthetic construct
  source 1..21: mol_type = other RNA
catttgttcagtggttcgtaa

SEQ ID NO: 285 - RNA, 21 nt, synthetic construct
  source 1..21: mol_type = other RNA
gggcgcacctctctttacgca

SEQ ID NO: 286 - RNA, 21 nt, synthetic construct
  source 1..21: mol_type = other RNA
tagactcgtggtggacttcta

SEQ ID NO: 287 - RNA, 21 nt, synthetic construct
  source 1..21: mol_type = other RNA
ggacttctctcaattttctaa

SEQ ID NO: 288 - RNA, 21 nt, synthetic construct
  source 1..21: mol_type = other RNA
ttggctcagtttactagtgca

SEQ ID NO: 289 - RNA, 21 nt, synthetic construct
  source 1..21: mol_type = other RNA
ctagtgccatttgttcagtga

SEQ ID NO: 290 - RNA, 21 nt, synthetic construct
  source 1..21: mol_type = other RNA
tgttaccaattttcttttgta

SEQ ID NO: 291 - RNA, 21 nt, synthetic construct
  source 1..21: mol_type = other RNA
ttcgcttcacctctgcacgta

SEQ ID NO: 292 - RNA, 21 nt, synthetic construct
  source 1..21: mol_type = other RNA
taggaggctgtaggcataaaa

SEQ ID NO: 293 - RNA, 21 nt, synthetic construct
  source 1..21: mol_type = other RNA
aggctgtaggcataaattgga

SEQ ID NO: 294 - RNA, 21 nt, synthetic construct
  source 1..21: mol_type = other RNA
cttctctcaattttctaggga

SEQ ID NO: 295 - RNA, 21 nt, synthetic construct
  source 1..21: mol_type = other RNA
ctgttaccaattttcttttga

SEQ ID NO: 296 - RNA, 21 nt, synthetic construct
  source 1..21: mol_type = other RNA
ccgtctgtgccttctcatcta

SEQ ID NO: 297 - RNA, 21 nt, synthetic construct
  source 1..21: mol_type = other RNA
tacataagaggactcttggaa

SEQ ID NO: 298 - RNA, 21 nt, synthetic construct
  source 1..21: mol_type = other RNA
tacaggcggggtttttcttga

SEQ ID NO: 299 - RNA, 21 nt, synthetic construct
  source 1..21: mol_type = other RNA
caggcggggtttttcttgtta

SEQ ID NO: 300 - RNA, 21 nt, synthetic construct
  source 1..21: mol_type = other RNA
cggggtttttcttgttgacaa

SEQ ID NO: 301 - RNA, 21 nt, synthetic construct
  source 1..21: mol_type = other RNA
ctcgtggtggacttctctcaa

SEQ ID NO: 302 - RNA, 21 nt, synthetic construct
  source 1..21: mol_type = other RNA
cgtggtggacttctctcaata

SEQ ID NO: 303 - RNA, 21 nt, synthetic construct
  source 1..21: mol_type = other RNA
gtggtggacttctctcaatta

SEQ ID NO: 304 - RNA, 21 nt, synthetic construct
  source 1..21: mol_type = other RNA
tttactagtgccatttgttca

SEQ ID NO: 305 - RNA, 21 nt, synthetic construct
  source 1..21: mol_type = other RNA
agtgccatttgttcagtggta

SEQ ID NO: 306 - RNA, 21 nt, synthetic construct
  source 1..21: mol_type = other RNA
ttaccaattttcttttgtcta

SEQ ID NO: 307 - RNA, 21 nt, synthetic construct
  source 1..21: mol_type = other RNA
aggcctattgattggaaagta

SEQ ID NO: 308 - RNA, 21 nt, synthetic construct
  source 1..21: mol_type = other RNA
ccgatccatactgcggaacta

SEQ ID NO: 309 - RNA, 21 nt, synthetic construct
  source 1..21: mol_type = other RNA
gtgtgcacttcgcttcaccta

SEQ ID NO: 310 - RNA, 21 nt, synthetic construct
  source 1..21: mol_type = other RNA
ttacataagaggactcttgga

SEQ ID NO: 311 - RNA, 21 nt, synthetic construct
  source 1..21: mol_type = other RNA
tcctgctgctatgcctcatca

SEQ ID NO: 312 - RNA, 21 nt, synthetic construct
  source 1..21: mol_type = other RNA
ctgtgccaagtgtttgctgaa

SEQ ID NO: 313 - RNA, 21 nt, synthetic construct
  source 1..21: mol_type = other RNA
tgtgccaagtgtttgctgaca

SEQ ID NO: 314 - RNA, 21 nt, synthetic construct
  source 1..21: mol_type = other RNA
cgtgtgcacttcgcttcacca

SEQ ID NO: 315 - RNA, 21 nt, synthetic construct
  source 1..21: mol_type = other RNA
gtataagaggactcttggaca

SEQ ID NO: 316 - RNA, 21 nt, synthetic construct
  source 1..21: mol_type = other RNA
gtctagactcgtggtggacta

SEQ ID NO: 317 - RNA, 21 nt, synthetic construct
  source 1..21: mol_type = other RNA
tctagactcgtggtggactta

SEQ ID NO: 318 - RNA, 21 nt, synthetic construct
  source 1..21: mol_type = other RNA
atcctgctgctatgcctcata

SEQ ID NO: 319 - RNA, 21 nt, synthetic construct
  source 1..21: mol_type = other RNA
aaggtatgttgcccgtttgta

SEQ ID NO: 320 - RNA, 21 nt, synthetic construct
  source 1..21: mol_type = other RNA
agtttactagtgccatttgta

SEQ ID NO: 321 - RNA, 21 nt, synthetic construct
  source 1..21: mol_type = other RNA
ccatttgttcagtggttcgta

SEQ ID NO: 322 - RNA, 21 nt, synthetic construct
  source 1..21: mol_type = other RNA
cagcgcatgcgtggaacctta

SEQ ID NO: 323 - RNA, 21 nt, synthetic construct
  source 1..21: mol_type = other RNA
atgtcaacgaccgaccttgaa

SEQ ID NO: 324 - RNA, 21 nt, synthetic construct
  source 1..21: mol_type = other RNA
gttacaggcggggtttttcta

SEQ ID NO: 325 - RNA, 21 nt, synthetic construct
  source 1..21: mol_type = other RNA
gcagagtctagactcgtggta

SEQ ID NO: 326 - RNA, 21 nt, synthetic construct
  source 1..21: mol_type = other RNA
gagtctagactcgtggtggaa

SEQ ID NO: 327 - RNA, 21 nt, synthetic construct
  source 1..21: mol_type = other RNA
cttcatcctgctgctatgcca

SEQ ID NO: 328 - RNA, 21 nt, synthetic construct
  source 1..21: mol_type = other RNA
cctgctgctatgcctcatcta

SEQ ID NO: 329 - RNA, 21 nt, synthetic construct
  source 1..21: mol_type = other RNA
aggtatgttgcccgtttgtca

SEQ ID NO: 330 - RNA, 21 nt, synthetic construct
  source 1..21: mol_type = other RNA
gtgccatttgttcagtggtta

SEQ ID NO: 331 - RNA, 21 nt, synthetic construct
  source 1..21: mol_type = other RNA
cggggcgcacctctctttaca

SEQ ID NO: 332 - RNA, 21 nt, synthetic construct
  source 1..21: mol_type = other RNA
ttacaggcggggtttttctta

SEQ ID NO: 333 - RNA, 21 nt, synthetic construct
  source 1..21: mol_type = other RNA
acaggcggggtttttcttgta

SEQ ID NO: 334 - RNA, 21 nt, synthetic construct
  source 1..21: mol_type = other RNA
tcaaggtatgttgcccgttta

SEQ ID NO: 335 - RNA, 21 nt, synthetic construct
  source 1..21: mol_type = other RNA
catactgcggaactcctagca

SEQ ID NO: 336 - RNA, 21 nt, synthetic construct
  source 1..21: mol_type = other RNA
gaccacggggcgcacctctca

SEQ ID NO: 337 - RNA, 21 nt, synthetic construct
  source 1..21: mol_type = other RNA
tgtcaacgaccgaccttgaga

SEQ ID NO: 338 - RNA, 21 nt, synthetic construct
  source 1..21: mol_type = other RNA
ttcatcctgctgctatgccta

SEQ ID NO: 339 - RNA, 21 nt, synthetic construct
  source 1..21: mol_type = other RNA
gctcctctgccgatccataca

SEQ ID NO: 340 - RNA, 21 nt, synthetic construct
  source 1..21: mol_type = other RNA
ctcctctgccgatccatacta

SEQ ID NO: 341 - RNA, 21 nt, synthetic construct
  source 1..21: mol_type = other RNA
cctctgccgatccatactgca

SEQ ID NO: 342 - RNA, 21 nt, synthetic construct
  source 1..21: mol_type = other RNA
cgatccatactgcggaactca

SEQ ID NO: 343 - RNA, 21 nt, synthetic construct
  source 1..21: mol_type = other RNA
ggcgcacctctctttacgcga

SEQ ID NO: 344 - RNA, 21 nt, synthetic construct
  source 1..21: mol_type = other RNA
cccgtctgtgccttctcatca

SEQ ID NO: 345 - RNA, 21 nt, synthetic construct
  source 1..21: mol_type = other RNA
tcaacgaccgaccttgaggca

SEQ ID NO: 346 - RNA, 19 nt, synthetic construct
  source 1..19: mol_type = other RNA
gtggacttctctcaattta

SEQ ID NO: 347 - RNA, 19 nt, synthetic construct
  source 1..19: mol_type = other RNA
ttctctcaattttctagga

SEQ ID NO: 348 - RNA, 19 nt, synthetic construct
  source 1..19: mol_type = other RNA
taccaattttcttttgtca

SEQ ID NO: 349 - RNA, 19 nt, synthetic construct
  source 1..19: mol_type = other RNA
taagaggactcttggacta

SEQ ID NO: 350 - RNA, 19 nt, synthetic construct
  source 1..19: mol_type = other RNA
ggtttttcttgttgacaaa

SEQ ID NO: 351 - RNA, 19 nt, synthetic construct
  source 1..19: mol_type = other RNA
gacttctctcaattttcta

SEQ ID NO: 352 - RNA, 19 nt, synthetic construct
  source 1..19: mol_type = other RNA
gctatgcctcatcttctta

SEQ ID NO: 353 - RNA, 19 nt, synthetic construct
  source 1..19: mol_type = other RNA
tttgttcagtggttcgtaa

SEQ ID NO: 354 - RNA, 19 nt, synthetic construct
  source 1..19: mol_type = other RNA
gcgcacctctctttacgca

SEQ ID NO: 355 - RNA, 19 nt, synthetic construct
  source 1..19: mol_type = other RNA
gactcgtggtggacttcta

SEQ ID NO: 356 - RNA, 19 nt, synthetic construct
  source 1..19: mol_type = other RNA
acttctctcaattttctaa

SEQ ID NO: 357 - RNA, 19 nt, synthetic construct
  source 1..19: mol_type = other RNA
ggctcagtttactagtgca

SEQ ID NO: 358 - RNA, 19 nt, synthetic construct
  source 1..19: mol_type = other RNA
agtgccatttgttcagtga

SEQ ID NO: 359 - RNA, 19 nt, synthetic construct
  source 1..19: mol_type = other RNA
ttaccaattttcttttgta

SEQ ID NO: 360 - RNA, 19 nt, synthetic construct
  source 1..19: mol_type = other RNA
cgcttcacctctgcacgta

SEQ ID NO: 361 - RNA, 19 nt, synthetic construct
  source 1..19: mol_type = other RNA
ggaggctgtaggcataaaa

SEQ ID NO: 362 - RNA, 19 nt, synthetic construct
  source 1..19: mol_type = other RNA
gctgtaggcataaattgga

SEQ ID NO: 363 - RNA, 19 nt, synthetic construct
  source 1..19: mol_type = other RNA
tctctcaattttctaggga

SEQ ID NO: 364 - RNA, 19 nt, synthetic construct
  source 1..19: mol_type = other RNA
gttaccaattttcttttga

SEQ ID NO: 365 - RNA, 19 nt, synthetic construct
  source 1..19: mol_type = other RNA
gtctgtgccttctcatcta

SEQ ID NO: 366 - RNA, 19 nt, synthetic construct
  source 1..19: mol_type = other RNA
cataagaggactcttggaa

SEQ ID NO: 367 - RNA, 19 nt, synthetic construct
  source 1..19: mol_type = other RNA
caggcggggtttttcttga

SEQ ID NO: 368 - RNA, 19 nt, synthetic construct
  source 1..19: mol_type = other RNA
ggcggggtttttcttgtta

SEQ ID NO: 369 - RNA, 19 nt, synthetic construct
  source 1..19: mol_type = other RNA
gggtttttcttgttgacaa

SEQ ID NO: 370 - RNA, 19 nt, synthetic construct
  source 1..19: mol_type = other RNA
cgtggtggacttctctcaa

SEQ ID NO: 371 - RNA, 19 nt, synthetic construct
  source 1..19: mol_type = other RNA
tggtggacttctctcaata

SEQ ID NO: 372 - RNA, 19 nt, synthetic construct
  source 1..19: mol_type = other RNA
ggtggacttctctcaatta

SEQ ID NO: 373 - RNA, 19 nt, synthetic construct
  source 1..19: mol_type = other RNA
tactagtgccatttgttca

SEQ ID NO: 374 - RNA, 19 nt, synthetic construct
  source 1..19: mol_type = other RNA
tgccatttgttcagtggta

SEQ ID NO: 375 - RNA, 19 nt, synthetic construct
  source 1..19: mol_type = other RNA
accaattttcttttgtcta

SEQ ID NO: 376 - RNA, 19 nt, synthetic construct
  source 1..19: mol_type = other RNA
gcctattgattggaaagta

SEQ ID NO: 377 - RNA, 19 nt, synthetic construct
  source 1..19: mol_type = other RNA
gatccatactgcggaacta

SEQ ID NO: 378 - RNA, 19 nt, synthetic construct
  source 1..19: mol_type = other RNA
gtgcacttcgcttcaccta

SEQ ID NO: 379 - RNA, 19 nt, synthetic construct
  source 1..19: mol_type = other RNA
acataagaggactcttgga

SEQ ID NO: 380 - RNA, 19 nt, synthetic construct
  source 1..19: mol_type = other RNA
ctgctgctatgcctcatca

SEQ ID NO: 381 - RNA, 19 nt, synthetic construct
  source 1..19: mol_type = other RNA
gtgccaagtgtttgctgaa

SEQ ID NO: 382 - RNA, 19 nt, synthetic construct
  source 1..19: mol_type = other RNA
tgccaagtgtttgctgaca

SEQ ID NO: 383 - RNA, 19 nt, synthetic construct
  source 1..19: mol_type = other RNA
tgtgcacttcgcttcacca

SEQ ID NO: 384 - RNA, 19 nt, synthetic construct
  source 1..19: mol_type = other RNA
ataagaggactcttggaca

SEQ ID NO: 385 - RNA, 19 nt, synthetic construct
  source 1..19: mol_type = other RNA
ctagactcgtggtggacta

SEQ ID NO: 386 - RNA, 19 nt, synthetic construct
  source 1..19: mol_type = other RNA
tagactcgtggtggactta

SEQ ID NO: 387 - RNA, 19 nt, synthetic construct
  source 1..19: mol_type = other RNA
cctgctgctatgcctcata

SEQ ID NO: 388 - RNA, 19 nt, synthetic construct
  source 1..19: mol_type = other RNA
ggtatgttgcccgtttgta

SEQ ID NO: 389 - RNA, 19 nt, synthetic construct
  source 1..19: mol_type = other RNA
tttactagtgccatttgta

SEQ ID NO: 390 - RNA, 19 nt, synthetic construct
  source 1..19: mol_type = other RNA
atttgttcagtggttcgta

SEQ ID NO: 391 - RNA, 19 nt, synthetic construct
  source 1..19: mol_type = other RNA
gcgcatgcgtggaacctta

SEQ ID NO: 392 - RNA, 19 nt, synthetic construct
  source 1..19: mol_type = other RNA
gtcaacgaccgaccttgaa

SEQ ID NO: 393 - RNA, 19 nt, synthetic construct
  source 1..19: mol_type = other RNA
tacaggcggggtttttcta

SEQ ID NO: 394 - RNA, 19 nt, synthetic construct
  source 1..19: mol_type = other RNA
agagtctagactcgtggta

SEQ ID NO: 395 - RNA, 19 nt, synthetic construct
  source 1..19: mol_type = other RNA
gtctagactcgtggtggaa

SEQ ID NO: 396 - RNA, 19 nt, synthetic construct
  source 1..19: mol_type = other RNA
tcatcctgctgctatgcca

SEQ ID NO: 397 - RNA, 19 nt, synthetic construct
  source 1..19: mol_type = other RNA
tgctgctatgcctcatcta

SEQ ID NO: 398 - RNA, 19 nt, synthetic construct
  source 1..19: mol_type = other RNA
gtatgttgcccgtttgtca

SEQ ID NO: 399 - RNA, 19 nt, synthetic construct
  source 1..19: mol_type = other RNA
gccatttgttcagtggtta

SEQ ID NO: 400 - RNA, 19 nt, synthetic construct
  source 1..19: mol_type = other RNA
gggcgcacctctctttaca

SEQ ID NO: 401 - RNA, 19 nt, synthetic construct
  source 1..19: mol_type = other RNA
acaggcggggtttttctta

SEQ ID NO: 402 - RNA, 19 nt, synthetic construct
  source 1..19: mol_type = other RNA
aggcggggtttttcttgta

SEQ ID NO: 403 - RNA, 19 nt, synthetic construct
  source 1..19: mol_type = other RNA
aaggtatgttgcccgttta

SEQ ID NO: 404 - RNA, 19 nt, synthetic construct
  source 1..19: mol_type = other RNA
tactgcggaactcctagca

SEQ ID NO: 405 - RNA, 19 nt, synthetic construct
  source 1..19: mol_type = other RNA
ccacggggcgcacctctca

SEQ ID NO: 406 - RNA, 19 nt, synthetic construct
  source 1..19: mol_type = other RNA
tcaacgaccgaccttgaga

SEQ ID NO: 407 - RNA, 19 nt, synthetic construct
  source 1..19: mol_type = other RNA
catcctgctgctatgccta

SEQ ID NO: 408 - RNA, 19 nt, synthetic construct
  source 1..19: mol_type = other RNA
tcctctgccgatccataca

SEQ ID NO: 409 - RNA, 19 nt, synthetic construct
  source 1..19: mol_type = other RNA
cctctgccgatccatacta

SEQ ID NO: 410 - RNA, 19 nt, synthetic construct
  source 1..19: mol_type = other RNA
tctgccgatccatactgca

SEQ ID NO: 411 - RNA, 19 nt, synthetic construct
  source 1..19: mol_type = other RNA
atccatactgcggaactca

SEQ ID NO: 412 - RNA, 19 nt, synthetic construct
  source 1..19: mol_type = other RNA
cgcacctctctttacgcga

SEQ ID NO: 413 - RNA, 19 nt, synthetic construct
  source 1..19: mol_type = other RNA
cgtctgtgccttctcatca

SEQ ID NO: 414 - RNA, 19 nt, synthetic construct
  source 1..19: mol_type = other RNA
aacgaccgaccttgaggca

SEQ ID NO: 415 - RNA, 21 nt, synthetic construct
  source 1..21: mol_type = other RNA
taaattgagagaagtccacca

SEQ ID NO: 416 - RNA, 21 nt, synthetic construct
  source 1..21: mol_type = other RNA
tcctagaaaattgagagaagt

SEQ ID NO: 417 - RNA, 21 nt, synthetic construct
  source 1..21: mol_type = other RNA
tgacaaaagaaaattggtaac

SEQ ID NO: 418 - RNA, 21 nt, synthetic construct
  source 1..21: mol_type = other RNA
tagtccaagagtcctcttatg

SEQ ID NO: 419 - RNA, 21 nt, synthetic construct
  source 1..21: mol_type = other RNA
tttgtcaacaagaaaaacccc

SEQ ID NO: 420 - RNA, 21 nt, synthetic construct
  source 1..21: mol_type = other RNA
tagaaaattgagagaagtcca

SEQ ID NO: 421 - RNA, 21 nt, synthetic construct
  source 1..21: mol_type = other RNA
taagaagatgaggcatagcag

SEQ ID NO: 422 - RNA, 21 nt, synthetic construct
  source 1..21: mol_type = other RNA
ttacgaaccactgaacaaatg

SEQ ID NO: 423 - RNA, 21 nt, synthetic construct
  source 1..21: mol_type = other RNA
tgcgtaaagagaggtgcgccc

SEQ ID NO: 424 - RNA, 21 nt, synthetic construct
  source 1..21: mol_type = other RNA
tagaagtccaccacgagtcta

SEQ ID NO: 425 - RNA, 21 nt, synthetic construct
  source 1..21: mol_type = other RNA
ttagaaaattgagagaagtcc

SEQ ID NO: 426 - RNA, 21 nt, synthetic construct
  source 1..21: mol_type = other RNA
tgcactagtaaactgagccaa

SEQ ID NO: 427 - RNA, 21 nt, synthetic construct
  source 1..21: mol_type = other RNA
tcactgaacaaatggcactag

SEQ ID NO: 428 - RNA, 21 nt, synthetic construct
  source 1..21: mol_type = other RNA
tacaaaagaaaattggtaaca

SEQ ID NO: 429 - RNA, 21 nt, synthetic construct
  source 1..21: mol_type = other RNA
tacgtgcagaggtgaagcgaa

SEQ ID NO: 430 - RNA, 21 nt, synthetic construct
  source 1..21: mol_type = other RNA
ttttatgcctacagcctccta

SEQ ID NO: 431 - RNA, 21 nt, synthetic construct
  source 1..21: mol_type = other RNA
tccaatttatgcctacagcct

SEQ ID NO: 432 - RNA, 21 nt, synthetic construct
  source 1..21: mol_type = other RNA
tccctagaaaattgagagaag

SEQ ID NO: 433 - RNA, 21 nt, synthetic construct
  source 1..21: mol_type = other RNA
tcaaaagaaaattggtaacag

SEQ ID NO: 434 - RNA, 21 nt, synthetic construct
  source 1..21: mol_type = other RNA
tagatgagaaggcacagacgg

SEQ ID NO: 435 - RNA, 21 nt, synthetic construct
  source 1..21: mol_type = other RNA
ttccaagagtcctcttatgta

SEQ ID NO: 436 - RNA, 21 nt, synthetic construct
  source 1..21: mol_type = other RNA
tcaagaaaaaccccgcctgta

SEQ ID NO: 437 - RNA, 21 nt, synthetic construct
  source 1..21: mol_type = other RNA
taacaagaaaaaccccgcctg

SEQ ID NO: 438 - RNA, 21 nt, synthetic construct
  source 1..21: mol_type = other RNA
ttgtcaacaagaaaaaccccg

SEQ ID NO: 439 - RNA, 21 nt, synthetic construct
  source 1..21: mol_type = other RNA
ttgagagaagtccaccacgag

SEQ ID NO: 440 - RNA, 21 nt, synthetic construct
  source 1..21: mol_type = other RNA
tattgagagaagtccaccacg

SEQ ID NO: 441 - RNA, 21 nt, synthetic construct
  source 1..21: mol_type = other RNA
taattgagagaagtccaccac

SEQ ID NO: 442 - RNA, 21 nt, synthetic construct
  source 1..21: mol_type = other RNA
tgaacaaatggcactagtaaa

SEQ ID NO: 443 - RNA, 21 nt, synthetic construct
  source 1..21: mol_type = other RNA
taccactgaacaaatggcact

SEQ ID NO: 444 - RNA, 21 nt, synthetic construct
  source 1..21: mol_type = other RNA
tagacaaaagaaaattggtaa

SEQ ID NO: 445 - RNA, 21 nt, synthetic construct
  source 1..21: mol_type = other RNA
tactttccaatcaataggcct

SEQ ID NO: 446 - RNA, 21 nt, synthetic construct
  source 1..21: mol_type = other RNA
tagttccgcagtatggatcgg

SEQ ID NO: 447 - RNA, 21 nt, synthetic construct
  source 1..21: mol_type = other RNA
taggtgaagcgaagtgcacac

SEQ ID NO: 448 - RNA, 21 nt, synthetic construct
  source 1..21: mol_type = other RNA
tccaagagtcctcttatgtaa

SEQ ID NO: 449 - RNA, 21 nt, synthetic construct
  source 1..21: mol_type = other RNA
tgatgaggcatagcagcagga

SEQ ID NO: 450 - RNA, 21 nt, synthetic construct
  source 1..21: mol_type = other RNA
ttcagcaaacacttggcacag

SEQ ID NO: 451 - RNA, 21 nt, synthetic construct
  source 1..21: mol_type = other RNA
tgtcagcaaacacttggcaca

SEQ ID NO: 452 - RNA, 21 nt, synthetic construct
  source 1..21: mol_type = other RNA
tggtgaagcgaagtgcacacg

SEQ ID NO: 453 - RNA, 21 nt, synthetic construct
  source 1..21: mol_type = other RNA
tgtccaagagtcctcttatac

SEQ ID NO: 454 - RNA, 21 nt, synthetic construct
  source 1..21: mol_type = other RNA
tagtccaccacgagtctagac

SEQ ID NO: 455 - RNA, 21 nt, synthetic construct
  source 1..21: mol_type = other RNA
taagtccaccacgagtctaga

SEQ ID NO: 456 - RNA, 21 nt, synthetic construct
  source 1..21: mol_type = other RNA
tatgaggcatagcagcaggat

SEQ ID NO: 457 - RNA, 21 nt, synthetic construct
  source 1..21: mol_type = other RNA
tacaaacgggcaacatacctt

SEQ ID NO: 458 - RNA, 21 nt, synthetic construct
  source 1..21: mol_type = other RNA
tacaaatggcactagtaaact

SEQ ID NO: 459 - RNA, 21 nt, synthetic construct
  source 1..21: mol_type = other RNA
tacgaaccactgaacaaatgg

SEQ ID NO: 460 - RNA, 21 nt, synthetic construct
  source 1..21: mol_type = other RNA
taaggttccacgcatgcgctg

SEQ ID NO: 461 - RNA, 21 nt, synthetic construct
  source 1..21: mol_type = other RNA
ttcaaggtcggtcgttgacat

SEQ ID NO: 462 - RNA, 21 nt, synthetic construct
  source 1..21: mol_type = other RNA
tagaaaaaccccgcctgtaac

SEQ ID NO: 463 - RNA, 21 nt, synthetic construct
  source 1..21: mol_type = other RNA
taccacgagtctagactctgc

SEQ ID NO: 464 - RNA, 21 nt, synthetic construct
  source 1..21: mol_type = other RNA
ttccaccacgagtctagactc

SEQ ID NO: 465 - RNA, 21 nt, synthetic construct
  source 1..21: mol_type = other RNA
tggcatagcagcaggatgaag

SEQ ID NO: 466 - RNA, 21 nt, synthetic construct
  source 1..21: mol_type = other RNA
tagatgaggcatagcagcagg

SEQ ID NO: 467 - RNA, 21 nt, synthetic construct
  source 1..21: mol_type = other RNA
tgacaaacgggcaacatacct

SEQ ID NO: 468 - RNA, 21 nt, synthetic construct
  source 1..21: mol_type = other RNA
taaccactgaacaaatggcac

SEQ ID NO: 469 - RNA, 21 nt, synthetic construct
  source 1..21: mol_type = other RNA
tgtaaagagaggtgcgccccg

SEQ ID NO: 470 - RNA, 21 nt, synthetic construct
  source 1..21: mol_type = other RNA
taagaaaaaccccgcctgtaa

SEQ ID NO: 471 - RNA, 21 nt, synthetic construct
  source 1..21: mol_type = other RNA
tacaagaaaaaccccgcctgt

SEQ ID NO: 472 - RNA, 21 nt, synthetic construct
  source 1..21: mol_type = other RNA
taaacgggcaacataccttga

SEQ ID NO: 473 - RNA, 21 nt, synthetic construct
  source 1..21: mol_type = other RNA
tgctaggagttccgcagtatg

SEQ ID NO: 474 - RNA, 21 nt, synthetic construct
  source 1..21: mol_type = other RNA
tgagaggtgcgccccgtggtc

SEQ ID NO: 475 - RNA, 21 nt, synthetic construct
  source 1..21: mol_type = other RNA
tctcaaggtcggtcgttgaca

SEQ ID NO: 476 - RNA, 21 nt, synthetic construct
  source 1..21: mol_type = other RNA
taggcatagcagcaggatgaa

SEQ ID NO: 477 - RNA, 21 nt, synthetic construct
  source 1..21: mol_type = other RNA
tgtatggatcggcagaggagc

SEQ ID NO: 478 - RNA, 21 nt, synthetic construct
  source 1..21: mol_type = other RNA
tagtatggatcggcagaggag

SEQ ID NO: 479 - RNA, 21 nt, synthetic construct
  source 1..21: mol_type = other RNA
tgcagtatggatcggcagagg

SEQ ID NO: 480 - RNA, 21 nt, synthetic construct
  source 1..21: mol_type = other RNA
tgagttccgcagtatggatcg

SEQ ID NO: 481 - RNA, 21 nt, synthetic construct
  source 1..21: mol_type = other RNA
tcgcgtaaagagaggtgcgcc

SEQ ID NO: 482 - RNA, 21 nt, synthetic construct
  source 1..21: mol_type = other RNA
tgatgagaaggcacagacggg

SEQ ID NO: 483 - RNA, 21 nt, synthetic construct
  source 1..21: mol_type = other RNA
tgcctcaaggtcggtcgttga

SEQ ID NO: 484 - RNA, 19 nt, synthetic construct
  source 1..19: mol_type = other RNA
taaattgagagaagtccac

SEQ ID NO: 485 - RNA, 19 nt, synthetic construct
  source 1..19: mol_type = other RNA
tcctagaaaattgagagaa

SEQ ID NO: 486 - RNA, 19 nt, synthetic construct
  source 1..19: mol_type = other RNA
tgacaaaagaaaattggta

SEQ ID NO: 487 - RNA, 19 nt, synthetic construct
  source 1..19: mol_type = other RNA
tagtccaagagtcctctta

SEQ ID NO: 488 - RNA, 19 nt, synthetic construct
  source 1..19: mol_type = other RNA
tttgtcaacaagaaaaacc

SEQ ID NO: 489 - RNA, 19 nt, synthetic construct
  source 1..19: mol_type = other RNA
tagaaaattgagagaagtc

SEQ ID NO: 490 - RNA, 19 nt, synthetic construct
  source 1..19: mol_type = other RNA
taagaagatgaggcatagc

SEQ ID NO: 491 - RNA, 19 nt, synthetic construct
  source 1..19: mol_type = other RNA
ttacgaaccactgaacaaa

SEQ ID NO: 492 - RNA, 19 nt, synthetic construct
  source 1..19: mol_type = other RNA
tgcgtaaagagaggtgcgc

SEQ ID NO: 493 - RNA, 19 nt, synthetic construct
  source 1..19: mol_type = other RNA
tagaagtccaccacgagtc

SEQ ID NO: 494 - RNA, 19 nt, synthetic construct
  source 1..19: mol_type = other RNA
ttagaaaattgagagaagt

SEQ ID NO: 495 - RNA, 19 nt, synthetic construct
  source 1..19: mol_type = other RNA
tgcactagtaaactgagcc

SEQ ID NO: 496 - RNA, 19 nt, synthetic construct
  source 1..19: mol_type = other RNA
tcactgaacaaatggcact

SEQ ID NO: 497 - RNA, 19 nt, synthetic construct
  source 1..19: mol_type = other RNA
tacaaaagaaaattggtaa

SEQ ID NO: 498 - RNA, 19 nt, synthetic construct
  source 1..19: mol_type = other RNA
tacgtgcagaggtgaagcg

SEQ ID NO: 499 - RNA, 19 nt, synthetic construct
  source 1..19: mol_type = other RNA
ttttatgcctacagcctcc

SEQ ID NO: 500 - RNA, 19 nt, synthetic construct
  source 1..19: mol_type = other RNA
tccaatttatgcctacagc

SEQ ID NO: 501 - RNA, 19 nt, synthetic construct
  source 1..19: mol_type = other RNA
tccctagaaaattgagaga

SEQ ID NO: 502 - RNA, 19 nt, synthetic construct
  source 1..19: mol_type = other RNA
tcaaaagaaaattggtaac

SEQ ID NO: 503 - RNA, 19 nt, synthetic construct
  source 1..19: mol_type = other RNA
tagatgagaaggcacagac

SEQ ID NO: 504 - RNA, 19 nt, synthetic construct
  source 1..19: mol_type = other RNA
ttccaagagtcctcttatg

SEQ ID NO: 505 - RNA, 19 nt, synthetic construct
  source 1..19: mol_type = other RNA
tcaagaaaaaccccgcctg

SEQ ID NO: 506 - RNA, 19 nt, synthetic construct
  source 1..19: mol_type = other RNA
taacaagaaaaaccccgcc

SEQ ID NO: 507 - RNA, 19 nt, synthetic construct
  source 1..19: mol_type = other RNA
ttgtcaacaagaaaaaccc

SEQ ID NO: 508 - RNA, 19 nt, synthetic construct
  source 1..19: mol_type = other RNA
ttgagagaagtccaccacg

SEQ ID NO: 509 - RNA, 19 nt, synthetic construct
  source 1..19: mol_type = other RNA
tattgagagaagtccacca

SEQ ID NO: 510 - RNA, 19 nt, synthetic construct
  source 1..19: mol_type = other RNA
taattgagagaagtccacc

SEQ ID NO: 511 - RNA, 19 nt, synthetic construct
  source 1..19: mol_type = other RNA
tgaacaaatggcactagta

SEQ ID NO: 512 - RNA, 19 nt, synthetic construct
  source 1..19: mol_type = other RNA
taccactgaacaaatggca

SEQ ID NO: 513 - RNA, 19 nt, synthetic construct
  source 1..19: mol_type = other RNA
tagacaaaagaaaattggt

SEQ ID NO: 514 - RNA, 19 nt, synthetic construct
  source 1..19: mol_type = other RNA
tactttccaatcaataggc

SEQ ID NO: 515 - RNA, 19 nt, synthetic construct
  source 1..19: mol_type = other RNA
tagttccgcagtatggatc

SEQ ID NO: 516 - RNA, 19 nt, synthetic construct
  source 1..19: mol_type = other RNA
taggtgaagcgaagtgcac

SEQ ID NO: 517 - RNA, 19 nt, synthetic construct
  source 1..19: mol_type = other RNA
tccaagagtcctcttatgt

SEQ ID NO: 518 - RNA, 19 nt, synthetic construct
  source 1..19: mol_type = other RNA
tgatgaggcatagcagcag

SEQ ID NO: 519 - RNA, 19 nt, synthetic construct
  source 1..19: mol_type = other RNA
ttcagcaaacacttggcac

SEQ ID NO: 520 - RNA, 19 nt, synthetic construct
  source 1..19: mol_type = other RNA
tgtcagcaaacacttggca

SEQ ID NO: 521 - RNA, 19 nt, synthetic construct
  source 1..19: mol_type = other RNA
tggtgaagcgaagtgcaca

SEQ ID NO: 522 - RNA, 19 nt, synthetic construct
  source 1..19: mol_type = other RNA
tgtccaagagtcctcttat

SEQ ID NO: 523 - RNA, 19 nt, synthetic construct
  source 1..19: mol_type = other RNA
tagtccaccacgagtctag

SEQ ID NO: 524 - RNA, 19 nt, synthetic construct
  source 1..19: mol_type = other RNA
taagtccaccacgagtcta

SEQ ID NO: 525 - RNA, 19 nt, synthetic construct
  source 1..19: mol_type = other RNA
tatgaggcatagcagcagg

SEQ ID NO: 526 - RNA, 19 nt, synthetic construct
  source 1..19: mol_type = other RNA
tacaaacgggcaacatacc

SEQ ID NO: 527 - RNA, 19 nt, synthetic construct
  source 1..19: mol_type = other RNA
tacaaatggcactagtaaa

SEQ ID NO: 528 - RNA, 19 nt, synthetic construct
  source 1..19: mol_type = other RNA
tacgaaccactgaacaaat

SEQ ID NO: 529 - RNA, 19 nt, synthetic construct
  source 1..19: mol_type = other RNA
taaggttccacgcatgcgc

SEQ ID NO: 530 - RNA, 19 nt, synthetic construct
  source 1..19: mol_type = other RNA
ttcaaggtcggtcgttgac

SEQ ID NO: 531 - RNA, 19 nt, synthetic construct
  source 1..19: mol_type = other RNA
tagaaaaaccccgcctgta

SEQ ID NO: 532 - RNA, 19 nt, synthetic construct
  source 1..19: mol_type = other RNA
taccacgagtctagactct

SEQ ID NO: 533 - RNA, 19 nt, synthetic construct
  source 1..19: mol_type = other RNA
ttccaccacgagtctagac

SEQ ID NO: 534 - RNA, 19 nt, synthetic construct
  source 1..19: mol_type = other RNA
tggcatagcagcaggatga

SEQ ID NO: 535 - RNA, 19 nt, synthetic construct
  source 1..19: mol_type = other RNA
tagatgaggcatagcagca

SEQ ID NO: 536 - RNA, 19 nt, synthetic construct
  source 1..19: mol_type = other RNA
tgacaaacgggcaacatac

SEQ ID NO: 537 - RNA, 19 nt, synthetic construct
  source 1..19: mol_type = other RNA
taaccactgaacaaatggc

SEQ ID NO: 538 - RNA, 19 nt, synthetic construct
  source 1..19: mol_type = other RNA
tgtaaagagaggtgcgccc

SEQ ID NO: 539 - RNA, 19 nt, synthetic construct
  source 1..19: mol_type = other RNA
taagaaaaaccccgcctgt

SEQ ID NO: 540 - RNA, 19 nt, synthetic construct
  source 1..19: mol_type = other RNA
tacaagaaaaaccccgcct

SEQ ID NO: 541 - RNA, 19 nt, synthetic construct
  source 1..19: mol_type = other RNA
taaacgggcaacatacctt

SEQ ID NO: 542 - RNA, 19 nt, synthetic construct
  source 1..19: mol_type = other RNA
tgctaggagttccgcagta

SEQ ID NO: 543 - RNA, 19 nt, synthetic construct
  source 1..19: mol_type = other RNA
tgagaggtgcgccccgtgg

SEQ ID NO: 544 - RNA, 19 nt, synthetic construct
  source 1..19: mol_type = other RNA
tctcaaggtcggtcgttga

SEQ ID NO: 545 - RNA, 19 nt, synthetic construct
  source 1..19: mol_type = other RNA
taggcatagcagcaggatg

SEQ ID NO: 546 - RNA, 19 nt, synthetic construct
  source 1..19: mol_type = other RNA
tgtatggatcggcagagga

SEQ ID NO: 547 - RNA, 19 nt, synthetic construct
  source 1..19: mol_type = other RNA
tagtatggatcggcagagg

SEQ ID NO: 548 - RNA, 19 nt, synthetic construct
  source 1..19: mol_type = other RNA
tgcagtatggatcggcaga

SEQ ID NO: 549 - RNA, 19 nt, synthetic construct
  source 1..19: mol_type = other RNA
tgagttccgcagtatggat

SEQ ID NO: 550 - RNA, 19 nt, synthetic construct
  source 1..19: mol_type = other RNA
tcgcgtaaagagaggtgcg

SEQ ID NO: 551 - RNA, 19 nt, synthetic construct
  source 1..19: mol_type = other RNA
tgatgagaaggcacagacg

SEQ ID NO: 552 - RNA, 19 nt, synthetic construct
  source 1..19: mol_type = other RNA
tgcctcaaggtcggtcgtt

SEQ ID NO: 553 - RNA, 21 nt, synthetic construct
  source 1..21: mol_type = other RNA
tggtggacttctctcaattta

SEQ ID NO: 554 - RNA, 21 nt, synthetic construct
  source 1..21: mol_type = other RNA
acttctctcaattttctagga

SEQ ID NO: 555 - RNA, 21 nt, synthetic construct
  source 1..21: mol_type = other RNA
gttaccaattttcttttgtca

SEQ ID NO: 556 - RNA, 21 nt, synthetic construct
  source 1..21: mol_type = other RNA
cataagaggactcttggacta

SEQ ID NO: 557 - RNA, 21 nt, synthetic construct
  source 1..21: mol_type = other RNA
ggggtttttcttgttgacaaa

SEQ ID NO: 558 - RNA, 21 nt, synthetic construct
  source 1..21: mol_type = other RNA
ttcgcttcacctctgcacgta

SEQ ID NO: 559 - RNA, 21 nt, synthetic construct
  source 1..21: mol_type = other RNA
ccgtctgtgccttctcatcta

SEQ ID NO: 560 - RNA, 21 nt, synthetic construct
  source 1..21: mol_type = other RNA
aggcctattgattggaaagta

SEQ ID NO: 561 - RNA, 21 nt, synthetic construct
  source 1..21: mol_type = other RNA
gtgtgcacttcgcttcaccta

SEQ ID NO: 562 - RNA, 21 nt, synthetic construct
  source 1..21: mol_type = other RNA
aggtatgttgcccgtttgtca

SEQ ID NO: 563 - RNA, 21 nt, synthetic construct
  source 1..21: mol_type = other RNA
cggggcgcacctctctttaca

SEQ ID NO: 564 - RNA, 21 nt, synthetic construct
  source 1..21: mol_type = other RNA
cccgtctgtgccttctcatca

SEQ ID NO: 565 - RNA, 21 nt, synthetic construct
  source 1..21: mol_type = other RNA
tggacttctctcaattttcta

SEQ ID NO: 566 - RNA, 21 nt, synthetic construct
  source 1..21: mol_type = other RNA
catttgttcagtggttcgtaa

SEQ ID NO: 567 - RNA, 21 nt, synthetic construct
  source 1..21: mol_type = other RNA
tgttaccaattttcttttgta

SEQ ID NO: 568 - RNA, 21 nt, synthetic construct
  source 1..21: mol_type = other RNA
aggctgtaggcataaattgga

SEQ ID NO: 569 - RNA, 21 nt, synthetic construct
  source 1..21: mol_type = other RNA
ctgttaccaattttcttttga

SEQ ID NO: 570 - RNA, 21 nt, synthetic construct
  source 1..21: mol_type = other RNA
tacaggcggggtttttcttga

SEQ ID NO: 571 - RNA, 21 nt, synthetic construct
  source 1..21: mol_type = other RNA
cggggtttttcttgttgacaa

SEQ ID NO: 572 - RNA, 21 nt, synthetic construct
  source 1..21: mol_type = other RNA
tttactagtgccatttgttca

SEQ ID NO: 573 - RNA, 21 nt, synthetic construct
  source 1..21: mol_type = other RNA
ttaccaattttcttttgtcta

SEQ ID NO: 574 - RNA, 21 nt, synthetic construct
  source 1..21: mol_type = other RNA
atcctgctgctatgcctcata

SEQ ID NO: 575 - RNA, 21 nt, synthetic construct
  source 1..21: mol_type = other RNA
cagcgcatgcgtggaacctta

SEQ ID NO: 576 - RNA, 21 nt, synthetic construct
  source 1..21: mol_type = other RNA
gctcctctgccgatccataca

SEQ ID NO: 577 - RNA, 21 nt, synthetic construct
  source 1..21: mol_type = other RNA
tacataagaggactcttggaa

SEQ ID NO: 578 - RNA, 21 nt, synthetic construct
  source 1..21: mol_type = other RNA
taaattgagagaagtccacca

SEQ ID NO: 579 - RNA, 21 nt, synthetic construct
  source 1..21: mol_type = other RNA
tcctagaaaattgagagaagt

SEQ ID NO: 580 - RNA, 21 nt, synthetic construct
  source 1..21: mol_type = other RNA
tgacaaaagaaaattggtaac

SEQ ID NO: 581 - RNA, 21 nt, synthetic construct
  source 1..21: mol_type = other RNA
tagtccaagagtcctcttatg

SEQ ID NO: 582 - RNA, 21 nt, synthetic construct
  source 1..21: mol_type = other RNA
tttgtcaacaagaaaaacccc

SEQ ID NO: 583 - RNA, 21 nt, synthetic construct
  source 1..21: mol_type = other RNA
tacgtgcagaggtgaagcgaa

SEQ ID NO: 584 - RNA, 21 nt, synthetic construct
  source 1..21: mol_type = other RNA
tagatgagaaggcacagacgg

SEQ ID NO: 585 - RNA, 21 nt, synthetic construct
  source 1..21: mol_type = other RNA
tactttccaatcaataggcct

SEQ ID NO: 586 - RNA, 21 nt, synthetic construct
  source 1..21: mol_type = other RNA
taggtgaagcgaagtgcacac

SEQ ID NO: 587 - RNA, 21 nt, synthetic construct
  source 1..21: mol_type = other RNA
tgacaaacgggcaacatacct

SEQ ID NO: 588 - RNA, 21 nt, synthetic construct
  source 1..21: mol_type = other RNA
tgtaaagagaggtgcgccccg

SEQ ID NO: 589 - RNA, 21 nt, synthetic construct
  source 1..21: mol_type = other RNA
tgatgagaaggcacagacggg

SEQ ID NO: 590 - RNA, 21 nt, synthetic construct
  source 1..21: mol_type = other RNA
tagaaaattgagagaagtcca

SEQ ID NO: 591 - RNA, 21 nt, synthetic construct
  source 1..21: mol_type = other RNA
ttacgaaccactgaacaaatg

SEQ ID NO: 592 - RNA, 21 nt, synthetic construct
  source 1..21: mol_type = other RNA
tacaaaagaaaattggtaaca

SEQ ID NO: 593 - RNA, 21 nt, synthetic construct
  source 1..21: mol_type = other RNA
tccaatttatgcctacagcct

SEQ ID NO: 594 - RNA, 21 nt, synthetic construct
  source 1..21: mol_type = other RNA
tcaaaagaaaattggtaacag

SEQ ID NO: 595 - RNA, 21 nt, synthetic construct
  source 1..21: mol_type = other RNA
tcaagaaaaaccccgcctgta

SEQ ID NO: 596 - RNA, 21 nt, synthetic construct
  source 1..21: mol_type = other RNA
ttgtcaacaagaaaaaccccg

SEQ ID NO: 597 - RNA, 21 nt, synthetic construct
  source 1..21: mol_type = other RNA
tgaacaaatggcactagtaaa

SEQ ID NO: 598 - RNA, 21 nt, synthetic construct
  source 1..21: mol_type = other RNA
tagacaaaagaaaattggtaa

SEQ ID NO: 599 - RNA, 21 nt, synthetic construct
  source 1..21: mol_type = other RNA
tatgaggcatagcagcaggat

SEQ ID NO: 600 - RNA, 21 nt, synthetic construct
  source 1..21: mol_type = other RNA
taaggttccacgcatgcgctg

SEQ ID NO: 601 - RNA, 21 nt, synthetic construct
  source 1..21: mol_type = other RNA
tgtatggatcggcagaggagc

SEQ ID NO: 602 - RNA, 21 nt, synthetic construct
  source 1..21: mol_type = other RNA
ttccaagagtcctcttatgta

SEQ ID NO: 603 - RNA, 21 nt, synthetic construct
  source 1..21: mol_type = other RNA
tggtggacttctctcaattta

SEQ ID NO: 604 - RNA, 21 nt, synthetic construct
  source 1..21: mol_type = other RNA
acttctctcaattttctagga

SEQ ID NO: 605 - RNA, 21 nt, synthetic construct
  source 1..21: mol_type = other RNA
gttaccaattttcttttgtca

SEQ ID NO: 606 - RNA, 21 nt, synthetic construct
  source 1..21: mol_type = other RNA
cataagaggactcttggacta

SEQ ID NO: 607 - RNA, 21 nt, synthetic construct
  source 1..21: mol_type = other RNA
ggggtttttcttgttgacaaa

SEQ ID NO: 608 - RNA, 21 nt, synthetic construct
  source 1..21: mol_type = other RNA
ttcgcttcacctctgcacgta

SEQ ID NO: 609 - RNA, 21 nt, synthetic construct
  source 1..21: mol_type = other RNA
ccgtctgtgccttctcatcta

SEQ ID NO: 610 - RNA, 21 nt, synthetic construct
  source 1..21: mol_type = other RNA
aggcctattgattggaaagta

SEQ ID NO: 611 - RNA, 21 nt, synthetic construct
  source 1..21: mol_type = other RNA
gtgtgcacttcgcttcaccta

SEQ ID NO: 612 - RNA, 21 nt, synthetic construct
  source 1..21: mol_type = other RNA
aggtatgttgcccgtttgtca

SEQ ID NO: 613 - RNA, 21 nt, synthetic construct
  source 1..21: mol_type = other RNA
cggggcgcacctctctttaca

SEQ ID NO: 614 - RNA, 21 nt, synthetic construct
  source 1..21: mol_type = other RNA
cccgtctgtgccttctcatca

SEQ ID NO: 615 - RNA, 21 nt, synthetic construct
  source 1..21: mol_type = other RNA
tggacttctctcaattttcta

SEQ ID NO: 616 - RNA, 21 nt, synthetic construct
  source 1..21: mol_type = other RNA
catttgttcagtggttcgtaa

SEQ ID NO: 617 - RNA, 21 nt, synthetic construct
  source 1..21: mol_type = other RNA
tgttaccaattttcttttgta

SEQ ID NO: 618 - RNA, 21 nt, synthetic construct
  source 1..21: mol_type = other RNA
aggctgtaggcataaattgga

SEQ ID NO: 619 - RNA, 21 nt, synthetic construct
  source 1..21: mol_type = other RNA
ctgttaccaattttcttttga

SEQ ID NO: 620 - RNA, 21 nt, synthetic construct
  source 1..21: mol_type = other RNA
tacaggcggggtttttcttga

SEQ ID NO: 621 - RNA, 21 nt, synthetic construct
  source 1..21: mol_type = other RNA
cggggtttttcttgttgacaa

SEQ ID NO: 622 - RNA, 21 nt, synthetic construct
  source 1..21: mol_type = other RNA
tttactagtgccatttgttca

SEQ ID NO: 623 - RNA, 21 nt, synthetic construct
  source 1..21: mol_type = other RNA
ttaccaattttcttttgtcta

SEQ ID NO: 624 - RNA, 21 nt, synthetic construct
  source 1..21: mol_type = other RNA
atcctgctgctatgcctcata

SEQ ID NO: 625 - RNA, 21 nt, synthetic construct
  source 1..21: mol_type = other RNA
cagcgcatgcgtggaacctta

SEQ ID NO: 626 - RNA, 21 nt, synthetic construct
  source 1..21: mol_type = other RNA
gctcctctgccgatccataca

SEQ ID NO: 627 - RNA, 21 nt, synthetic construct
  source 1..21: mol_type = other RNA
tacataagaggactcttggaa

SEQ ID NO: 628 - RNA, 21 nt, synthetic construct
  source 1..21: mol_type = other RNA
cgggtttttcttgttgacaaa

SEQ ID NO: 629 - RNA, 21 nt, synthetic construct
  source 1..21: mol_type = other RNA
cgttaccaattttcttttgta

SEQ ID NO: 630 - RNA, 21 nt, synthetic construct
  source 1..21: mol_type = other RNA
gtgttaccaattttcttttga

SEQ ID NO: 631 - RNA, 21 nt, synthetic construct
  source 1..21: mol_type = other RNA
cagggtttttcttgttgacat

SEQ ID NO: 632 - RNA, 21 nt, synthetic construct
  source 1..21: mol_type = other RNA
cttactagtgccatttgttca

SEQ ID NO: 633 - RNA, 21 nt, synthetic construct
  source 1..21: mol_type = other RNA
ctaccaattttcttttgtcta

SEQ ID NO: 634 - RNA, 21 nt, synthetic construct
  source 1..21: mol_type = other RNA
cggcctattgattggaaagta

SEQ ID NO: 635 - RNA, 21 nt, synthetic construct
  source 1..21: mol_type = other RNA
cagggcgcacctctctttaca

SEQ ID NO: 636 - RNA, 21 nt, synthetic construct
  source 1..21: mol_type = other RNA
aggggtttttcttgttgacat

SEQ ID NO: 637 - RNA, 21 nt, synthetic construct
  source 1..21: mol_type = other RNA
cgaggtttttcttgttgacaa

SEQ ID NO: 638 - RNA, 21 nt, synthetic construct
  source 1..21: mol_type = other RNA
taaattgagagaagtccacca

SEQ ID NO: 639 - RNA, 21 nt, synthetic construct
  source 1..21: mol_type = other RNA
tcctagaaaattgagagaagt

SEQ ID NO: 640 - RNA, 21 nt, synthetic construct
  source 1..21: mol_type = other RNA
tgacaaaagaaaattggtaac

SEQ ID NO: 641 - RNA, 21 nt, synthetic construct
  source 1..21: mol_type = other RNA
tagtccaagagtcctcttatg

SEQ ID NO: 642 - RNA, 21 nt, synthetic construct
  source 1..21: mol_type = other RNA
tttgtcaacaagaaaaacccc

SEQ ID NO: 643 - RNA, 21 nt, synthetic construct
  source 1..21: mol_type = other RNA
tacgtgcagaggtgaagcgaa

SEQ ID NO: 644 - RNA, 21 nt, synthetic construct
  source 1..21: mol_type = other RNA
tagatgagaaggcacagacgg

SEQ ID NO: 645 - RNA, 21 nt, synthetic construct
  source 1..21: mol_type = other RNA
tactttccaatcaataggcct

SEQ ID NO: 646 - RNA, 21 nt, synthetic construct
  source 1..21: mol_type = other RNA
taggtgaagcgaagtgcacac

SEQ ID NO: 647 - RNA, 21 nt, synthetic construct
  source 1..21: mol_type = other RNA
tgacaaacgggcaacatacct

SEQ ID NO: 648 - RNA, 21 nt, synthetic construct
  source 1..21: mol_type = other RNA
tgtaaagagaggtgcgccccg

SEQ ID NO: 649 - RNA, 21 nt, synthetic construct
  source 1..21: mol_type = other RNA
tgatgagaaggcacagacggg

SEQ ID NO: 650 - RNA, 21 nt, synthetic construct
  source 1..21: mol_type = other RNA
tagaaaattgagagaagtcca

SEQ ID NO: 651 - RNA, 21 nt, synthetic construct
  source 1..21: mol_type = other RNA
ttacgaaccactgaacaaatg

SEQ ID NO: 652 - RNA, 21 nt, synthetic construct
  source 1..21: mol_type = other RNA
tacaaaagaaaattggtaaca

SEQ ID NO: 653 - RNA, 21 nt, synthetic construct
  source 1..21: mol_type = other RNA
tccaatttatgcctacagcct

SEQ ID NO: 654 - RNA, 21 nt, synthetic construct
  source 1..21: mol_type = other RNA
tcaaaagaaaattggtaacag

SEQ ID NO: 655 - RNA, 21 nt, synthetic construct
  source 1..21: mol_type = other RNA
tcaagaaaaaccccgcctgta

SEQ ID NO: 656 - RNA, 21 nt, synthetic construct
  source 1..21: mol_type = other RNA
ttgtcaacaagaaaaaccccg

SEQ ID NO: 657 - RNA, 21 nt, synthetic construct
  source 1..21: mol_type = other RNA
tgaacaaatggcactagtaaa

SEQ ID NO: 658 - RNA, 21 nt, synthetic construct
  source 1..21: mol_type = other RNA
tagacaaaagaaaattggtaa

SEQ ID NO: 659 - RNA, 21 nt, synthetic construct
  source 1..21: mol_type = other RNA
tatgaggcatagcagcaggat

SEQ ID NO: 660 - RNA, 21 nt, synthetic construct
  source 1..21: mol_type = other RNA
taaggttccacgcatgcgctg

SEQ ID NO: 661 - RNA, 21 nt, synthetic construct
  source 1..21: mol_type = other RNA
tgtatggatcggcagaggagc

SEQ ID NO: 662 - RNA, 21 nt, synthetic construct
  source 1..21: mol_type = other RNA
ttccaagagtcctcttatgta

SEQ ID NO: 663 - RNA, 21 nt, synthetic construct
  source 1..21: mol_type = other RNA
tttgtcaacaagaaaaacccg

SEQ ID NO: 664 - RNA, 21 nt, synthetic construct
  source 1..21: mol_type = other RNA
tacaaaagaaaattggtaacg

SEQ ID NO: 665 - RNA, 21 nt, synthetic construct
  source 1..21: mol_type = other RNA
tcaaaagaaaattggtaacac

SEQ ID NO: 666 - RNA, 21 nt, synthetic construct
  source 1..21: mol_type = other RNA
atgtcaacaagaaaaaccctg

SEQ ID NO: 667 - RNA, 21 nt, synthetic construct
  source 1..21: mol_type = other RNA
tgaacaaatggcactagtaag

SEQ ID NO: 668 - RNA, 21 nt, synthetic construct
  source 1..21: mol_type = other RNA
tagacaaaagaaaattggtag

SEQ ID NO: 669 - RNA, 21 nt, synthetic construct
  source 1..21: mol_type = other RNA
tactttccaatcaataggccg

SEQ ID NO: 670 - RNA, 21 nt, synthetic construct
  source 1..21: mol_type = other RNA
tgtaaagagaggtgcgccctg

SEQ ID NO: 671 - RNA, 21 nt, synthetic construct
  source 1..21: mol_type = other RNA
atgtcaacaagaaaaacccct

SEQ ID NO: 672 - RNA, 21 nt, synthetic construct
  source 1..21: mol_type = other RNA
ttgtcaacaagaaaaacctcg

SEQ ID NO: 673 - RNA, 3221 nt, Homo sapiens
  source 1..3221: mol_type = mRNA
ttccactgccttccaccaagctctgcaggatcccaaagtcaggggtctgtattttcctgctggtggctccagttcaggaacagtaaaccctgctccgaatattgcctctcacatctcgtcaatctccgcgaggactggggaccctgtgacgaatatggagaacatcacatcaggattcctaggacccctgctcgtgttacaggcggggtttttcttgttgacaagaatcctcacaataccgcagagtctagactcgtggtggacttctctcaattttctagggggatcacccgtgtgtcttggccaaaattcgcagtccccaacctccaatcactcaccaacctcctgtcctccaatttgtcctggttatcgctggatgtgtctgcggcgttttatcatattcctcttcatcctgctgctatgcctcatcttcttgttggttcttctggattatcaaggtatgttgcccgtttgtcctctaattccaggaacaacaacaaccagtacgggaccatgcaaaacctgcacgactcctgctcaaggcaactctatgtttccctcatgttgctgtacaaaaccttcggatggaaattgcacctgtattcccatcccatcgtcttgggctttcgcaaaatacctatgggagtgggcctcagtccgtttctcttggctcagtttactagtgccatttgttcagtggttcgtagggctttcccccactgtttggctttcagctatatggatgatgtggtattgggggccaagtctgtacagcatcgtgagtccctttataccgctgttaccaattttcttttgtctctgggtatacatttaaaccctaacaaaacaaaaagatggggttattccctaaacttcatgggttacataattggaagttggggaacgttgccacaggatcatattgtacaaaagatcaaacactgttttagaaaacttcctgttaacaggcctattgattggaaagtatgtcaaagaattgtgggtcttttgggctttgctgctccatttacacaatgtggatatcctgccttaatgcctttgtatgcctgtatacaagctaaacaggctttcactttctcgccaacttacaaggcctttctaagtaaacagtacatgaacctttaccccgttgctcggcaacggcctggtctgtgccaagtgtttgctgacgcaacccccactggctggggcttggccataggccatcagcgcatgcgtggaacctttgtggctcctctgccgatccatactgcggaactcctagccgcttgttttgctcgcagccggtctggggcaaagctcatcggaactgacaattctgtcgtcctctcgcggaaatatacatcgtttccatggctgctaggttgtactgccaactggatccttcgcgggacgtcctttgtttacgtcccgtcggcgctgaatcccgcggacgacccctctcggggccgcttgggactctctcgtccccttctccgtctgccgttccagccgaccacggggcgcacctctctttacgcggtctccccgtctgtgccttctcatctgccggtccgtgtgcacttcgcttcacctctgcacgttgcatggagaccaccgtgaacgcccatcagatcctgcccaaggtcttacataagaggactcttggactcccagcaatgtcaacgaccgaccttgaggcctacttcaaagactgtgtgtttaaggactgggaggagctgggggaggagattaggttaaaggtctttgtattaggaggctgtaggcataaattggtctgcgcaccagcaccatgcaactttttcacctctgcctaatcatctcttgtacatgtcccactgttcaagcctccaagctgtgccttgggtggctttggggcatggacattgacccttataaagaatttggagctactgtggagttactctcgtttttgccttctgacttttttccttccgtcagagatctcctagacaccgcctcagctctgtatcgggaagccttagagtctcctgagcattgctcacctcaccatactgcactcaggcaagcaattctctgctggggggaattgatgactctagctacctgggtgggtaataatttggaagatccagcatccagggatctagtagtcaattatgttaatactaacatgggtttaaagatcaggcaactattgtggtttcatatatcttgccttacttttggaagagagactgtacttgaatatttggtctctttcggagtgtggattcgcactcctccagcctatagaccaccaaatgcccctatcttatcaacacttccggaaactactgttgttagacgacgggaccgaggcaggtcccctagaagaagaactccctcgcctcgcagacgcagatctcaatcgccgcgtcgcagaagatctcaatctcgggaatctcaatgttagtattccttggactcataaggtgggaaactttactgggctttattcctctacagtacctatctttaatcctgaatggcaaactccttcctttcctaagattcatttacaagaggacattattaataggtgtcaacaatttgtgggccctctcactgtaaatgaaaagagaagattgaaattaattatgcctgctagattctatcctacccacactaaatatttgcccttagacaaaggaattaaaccttattatccagatcaggtagttaatcattacttcaaaaccagacattatttacatactctttggaaggctggtattctatataagagggaaaccacacgtagcgcatcattttgcgggtcaccatattcttgggaacaagagctacagcatgggaggttggtcatcgaaacctcgcaaaggcatggggacgaatctttctgttcccaaccctctgggattctttcccgatcatcagttggaccctgcattcggagccaactcaaacaatccagattgggacttcaaccccatcaaggaccactggccagcagccaaccaggtaggagtgggagcattcgggccagggttcacccctccacacggcggtgttttggggtggagccctcaggctcagggcatattgaccacagtgtcaacaattcctcctcctgcctccaccaatcggcagtcaggaaggcagcctactcccatctctccacctctaagagacagtcatcctcaggccatgcagtggaa

SEQ ID NO: 674 - RNA, 21 nt, synthetic construct
  source 1..21: mol_type = other RNA
cgggtttttcttgttgacaaa

SEQ ID NO: 675 - RNA, 21 nt, synthetic construct
  source 1..21: mol_type = other RNA
cgggtttttcttgttgacaat

SEQ ID NO: 676 - RNA, 21 nt, synthetic construct
  source 1..21: mol_type = other RNA
cgggtttttcttgttgacaac

SEQ ID NO: 677 - RNA, 21 nt, synthetic construct
  source 1..21: mol_type = other RNA
cgggtttttcttgttgacaag

SEQ ID NO: 678 - RNA, 17 nt, synthetic construct
  source 1..17: mol_type = other RNA
tttttcttgttgacaaa

SEQ ID NO: 679 - RNA, 18 nt, synthetic construct
  source 1..18: mol_type = other RNA
gtttttcttgttgacaaa

SEQ ID NO: 680 - RNA, 19 nt, synthetic construct
  source 1..19: mol_type = other RNA
agtttttcttgttgacaaa

SEQ ID NO: 681 - RNA, 19 nt, synthetic construct
  source 1..19: mol_type = other RNA
tgtttttcttgttgacaaa

SEQ ID NO: 682 - RNA, 19 nt, synthetic construct
  source 1..19: mol_type = other RNA
ggtttttcttgttgacaaa

SEQ ID NO: 683 - RNA, 19 nt, synthetic construct
  source 1..19: mol_type = other RNA
cgtttttcttgttgacaaa

SEQ ID NO: 684 - RNA, 20 nt, synthetic construct
  source 1..20: mol_type = other RNA
aggtttttcttgttgacaaa

SEQ ID NO: 685 - RNA, 20 nt, synthetic construct
  source 1..20: mol_type = other RNA
tggtttttcttgttgacaaa

SEQ ID NO: 686 - RNA, 20 nt, synthetic construct
  source 1..20: mol_type = other RNA
gggtttttcttgttgacaaa

SEQ ID NO: 687 - RNA, 20 nt, synthetic construct
  source 1..20: mol_type = other RNA
cggtttttcttgttgacaaa

SEQ ID NO: 688 - RNA, 21 nt, synthetic construct
  source 1..21: mol_type = other RNA
agggtttttcttgttgacaaa

SEQ ID NO: 689 - RNA, 21 nt, synthetic construct
  source 1..21: mol_type = other RNA
tgggtttttcttgttgacaaa

SEQ ID NO: 690 - RNA, 22 nt, synthetic construct
  source 1..22: mol_type = other RNA
cggggtttttcttgttgacaaa

SEQ ID NO: 691 - RNA, 23 nt, synthetic construct
  source 1..23: mol_type = other RNA
gcggggtttttcttgttgacaaa

SEQ ID NO: 692 - RNA, 24 nt, synthetic construct
  source 1..24: mol_type = other RNA
ggcggggtttttcttgttgacaaa

SEQ ID NO: 693 - RNA, 25 nt, synthetic construct
  source 1..25: mol_type = other RNA
aggcggggtttttcttgttgacaaa

SEQ ID NO: 694 - RNA, 26 nt, synthetic construct
  source 1..26: mol_type = other RNA
caggcggggtttttcttgttgacaaa

SEQ ID NO: 695 - RNA, 32 nt, synthetic construct
  source 1..32: mol_type = other RNA
gtgttacaggcggggtttttcttgttgacaaa

SEQ ID NO: 696 - RNA, 21 nt, synthetic construct
  source 1..21: mol_type = other RNA
cgggtttttcttgttgacaaa

SEQ ID NO: 697 - RNA, 21 nt, synthetic construct
  source 1..21: mol_type = other RNA
cgggtttttcttgttgacaaa

SEQ ID NO: 698 - RNA, 21 nt, synthetic construct
  source 1..21: mol_type = other RNA
cgggtttttcttgttgacaaa

SEQ ID NO: 699 - RNA, 21 nt, synthetic construct
  source 1..21: mol_type = other RNA
cgggtttttcttgttgacaaa

SEQ ID NO: 700 - RNA, 21 nt, synthetic construct
  source 1..21: mol_type = other RNA
cgggtttttcttgttgacaaa

SEQ ID NO: 701 - RNA, 21 nt, synthetic construct
  source 1..21: mol_type = other RNA
cgggtttttcttgttaacaaa

SEQ ID NO: 702 - RNA, 21 nt, synthetic construct
  source 1..21: mol_type = other RNA
cgggtttttcttgttgacaga

SEQ ID NO: 703 - RNA, 21 nt, synthetic construct
  source 1..21: mol_type = other RNA
cgggtttttcttgttgacaaa

SEQ ID NO: 704 - RNA, 21 nt, synthetic construct
  source 1..21: mol_type = other RNA
cagggtttttcttgttgacat

SEQ ID NO: 705 - RNA, 21 nt, synthetic construct
  source 1..21: mol_type = other RNA
cagggtttttcttgttgacaa

SEQ ID NO: 706 - RNA, 21 nt, synthetic construct
  source 1..21: mol_type = other RNA
cagggtttttcttgttgacac

SEQ ID NO: 707 - RNA, 21 nt, synthetic construct
  source 1..21: mol_type = other RNA
cagggtttttcttgttgacag

SEQ ID NO: 708 - RNA, 17 nt, synthetic construct
  source 1..17: mol_type = other RNA
gtttttcttgttgacat

SEQ ID NO: 709 - RNA, 18 nt, synthetic construct
  source 1..18: mol_type = other RNA
ggtttttcttgttgacat

SEQ ID NO: 710 - RNA, 19 nt, synthetic construct
  source 1..19: mol_type = other RNA
aggtttttcttgttgacat

SEQ ID NO: 711 - RNA, 19 nt, synthetic construct
  source 1..19: mol_type = other RNA
tggtttttcttgttgacat

SEQ ID NO: 712 - RNA, 19 nt, synthetic construct
  source 1..19: mol_type = other RNA
gggtttttcttgttgacat

SEQ ID NO: 713 - RNA, 19 nt, synthetic construct
  source 1..19: mol_type = other RNA
cggtttttcttgttgacat

SEQ ID NO: 714 - RNA, 20 nt, synthetic construct
  source 1..20: mol_type = other RNA
agggtttttcttgttgacat

SEQ ID NO: 715 - RNA, 20 nt, synthetic construct
  source 1..20: mol_type = other RNA
tgggtttttcttgttgacat

SEQ ID NO: 716 - RNA, 20 nt, synthetic construct
  source 1..20: mol_type = other RNA
ggggtttttcttgttgacat

SEQ ID NO: 717 - RNA, 20 nt, synthetic construct
  source 1..20: mol_type = other RNA
cgggtttttcttgttgacat

SEQ ID NO: 718 - RNA, 21 nt, synthetic construct
  source 1..21: mol_type = other RNA
gagggtttttcttgttgacat

SEQ ID NO: 719 - RNA, 21 nt, synthetic construct
  source 1..21: mol_type = other RNA
aagggtttttcttgttgacat

SEQ ID NO: 720 - RNA, 21 nt, synthetic construct
  source 1..21: mol_type = other RNA
tagggtttttcttgttgacat

SEQ ID NO: 721 - RNA, 22 nt, synthetic construct
  source 1..22: mol_type = other RNA
gcggggtttttcttgttgacat

SEQ ID NO: 722 - RNA, 23 nt, synthetic construct
  source 1..23: mol_type = other RNA
ggcggggtttttcttgttgacat

SEQ ID NO: 723 - RNA, 24 nt, synthetic construct
  source 1..24: mol_type = other RNA
aggcggggtttttcttgttgacat

SEQ ID NO: 724 - RNA, 25 nt, synthetic construct
  source 1..25: mol_type = other RNA
caggcggggtttttcttgttgacat

SEQ ID NO: 725 - RNA, 26 nt, synthetic construct
  source 1..26: mol_type = other RNA
acaggcggggtttttcttgttgacat

SEQ ID NO: 726 - RNA, 32 nt, synthetic construct
  source 1..32: mol_type = other RNA
cgtgttacaggcggggtttttcttgttgacat

SEQ ID NO: 727 - RNA, 21 nt, synthetic construct
  source 1..21: mol_type = other RNA
cagggtttttcttgttgacat

SEQ ID NO: 728 - RNA, 21 nt, synthetic construct
  source 1..21: mol_type = other RNA
cagggtttttcttgttgacat

SEQ ID NO: 729 - RNA, 21 nt, synthetic construct
  source 1..21: mol_type = other RNA
cagggtttttcttgttgacat

SEQ ID NO: 730 - RNA, 21 nt, synthetic construct
  source 1..21: mol_type = other RNA
cagggtttttcttgttgacat

SEQ ID NO: 731 - RNA, 21 nt, synthetic construct
  source 1..21: mol_type = other RNA
cagggtttttcttgttgacat

SEQ ID NO: 732 - RNA, 21 nt, synthetic construct
  source 1..21: mol_type = other RNA
cagggtttttcttgtcgacat

SEQ ID NO: 733 - RNA, 21 nt, synthetic construct
  source 1..21: mol_type = other RNA
cagggtttttcttgttgacgt

SEQ ID NO: 734 - RNA, 21 nt, synthetic construct
  source 1..21: mol_type = other RNA
cagggtttttcttgttgacat

SEQ ID NO: 735 - RNA, 21 nt, synthetic construct
  source 1..21: mol_type = other RNA
tttgtcaacaagaaaaacccg

SEQ ID NO: 736 - RNA, 21 nt, synthetic construct
  source 1..21: mol_type = other RNA
attgtcaacaagaaaaacccg

SEQ ID NO: 737 - RNA, 21 nt, synthetic construct
  source 1..21: mol_type = other RNA
gttgtcaacaagaaaaacccg

SEQ ID NO: 738 - RNA, 21 nt, synthetic construct
  source 1..21: mol_type = other RNA
cttgtcaacaagaaaaacccg

SEQ ID NO: 739 - RNA, 17 nt, synthetic construct
  source 1..17: mol_type = other RNA
tttgtcaacaagaaaaa

SEQ ID NO: 740 - RNA, 18 nt, synthetic construct
  source 1..18: mol_type = other RNA
tttgtcaacaagaaaaac

SEQ ID NO: 741 - RNA, 19 nt, synthetic construct
  source 1..19: mol_type = other RNA
tttgtcaacaagaaaaact

SEQ ID NO: 742 - RNA, 19 nt, synthetic construct
  source 1..19: mol_type = other RNA
tttgtcaacaagaaaaaca

SEQ ID NO: 743 - RNA, 19 nt, synthetic construct
  source 1..19: mol_type = other RNA
tttgtcaacaagaaaaacc

SEQ ID NO: 744 - RNA, 19 nt, synthetic construct
  source 1..19: mol_type = other RNA
tttgtcaacaagaaaaacg

SEQ ID NO: 745 - RNA, 20 nt, synthetic construct
  source 1..20: mol_type = other RNA
tttgtcaacaagaaaaacct

SEQ ID NO: 746 - RNA, 20 nt, synthetic construct
  source 1..20: mol_type = other RNA
tttgtcaacaagaaaaacca

SEQ ID NO: 747 - RNA, 20 nt, synthetic construct
  source 1..20: mol_type = other RNA
tttgtcaacaagaaaaaccc

SEQ ID NO: 748 - RNA, 20 nt, synthetic construct
  source 1..20: mol_type = other RNA
tttgtcaacaagaaaaaccg

SEQ ID NO: 749 - RNA, 21 nt, synthetic construct
  source 1..21: mol_type = other RNA
tttgtcaacaagaaaaaccct

SEQ ID NO: 750 - RNA, 21 nt, synthetic construct
  source 1..21: mol_type = other RNA
tttgtcaacaagaaaaaccca

SEQ ID NO: 751 - RNA, 22 nt, synthetic construct
  source 1..22: mol_type = other RNA
tttgtcaacaagaaaaaccccg

SEQ ID NO: 752 - RNA, 23 nt, synthetic construct
  source 1..23: mol_type = other RNA
tttgtcaacaagaaaaaccccgc

SEQ ID NO: 753 - RNA, 24 nt, synthetic construct
  source 1..24: mol_type = other RNA
tttgtcaacaagaaaaaccccgcc

SEQ ID NO: 754 - RNA, 25 nt, synthetic construct
  source 1..25: mol_type = other RNA
tttgtcaacaagaaaaaccccgcct

SEQ ID NO: 755 - RNA, 26 nt, synthetic construct
  source 1..26: mol_type = other RNA
tttgtcaacaagaaaaaccccgcctg

SEQ ID NO: 756 - RNA, 32 nt, synthetic construct
  source 1..32: mol_type = other RNA
tttgtcaacaagaaaaaccccgcctgtaacac

SEQ ID NO: 757 - RNA, 23 nt, synthetic construct
  source 1..23: mol_type = other RNA
tttgtcaacaagaaaaacccgtt

SEQ ID NO: 758 - RNA, 23 nt, synthetic construct
  source 1..23: mol_type = other RNA
tttgtcaacaagaaaaacccgga

SEQ ID NO: 759 - RNA, 21 nt, synthetic construct
  source 1..21: mol_type = other RNA
tttgtcaacaagaaaaacccg

SEQ ID NO: 760 - RNA, 21 nt, synthetic construct
  source 1..21: mol_type = other RNA
tttgtcaacaagaaaaacccg

SEQ ID NO: 761 - RNA, 21 nt, synthetic construct
  source 1..21: mol_type = other RNA
tttgtcaacaagaaaaacccg

SEQ ID NO: 762 - RNA, 21 nt, synthetic construct
  source 1..21: mol_type = other RNA
tttgtcaacaagaaaaacccg

SEQ ID NO: 763 - RNA, 21 nt, synthetic construct
  source 1..21: mol_type = other RNA
tctgtcaacaagaaaaacccg

SEQ ID NO: 764 - RNA, 21 nt, synthetic construct
  source 1..21: mol_type = other RNA
tttgtcaacaagaaaaacccg

SEQ ID NO: 765 - RNA, 21 nt, synthetic construct
  source 1..21: mol_type = other RNA
atgtcaacaagaaaaaccctg

SEQ ID NO: 766 - RNA, 21 nt, synthetic construct
  source 1..21: mol_type = other RNA
ttgtcaacaagaaaaaccctg

SEQ ID NO: 767 - RNA, 21 nt, synthetic construct
  source 1..21: mol_type = other RNA
gtgtcaacaagaaaaaccctg

SEQ ID NO: 768 - RNA, 21 nt, synthetic construct
  source 1..21: mol_type = other RNA
ctgtcaacaagaaaaaccctg

SEQ ID NO: 769 - RNA, 17 nt, synthetic construct
  source 1..17: mol_type = other RNA
atgtcaacaagaaaaac

SEQ ID NO: 770 - RNA, 18 nt, synthetic construct
  source 1..18: mol_type = other RNA
atgtcaacaagaaaaacc

SEQ ID NO: 771 - RNA, 19 nt, synthetic construct
  source 1..19: mol_type = other RNA
atgtcaacaagaaaaacct

SEQ ID NO: 772 - RNA, 19 nt, synthetic construct
  source 1..19: mol_type = other RNA
atgtcaacaagaaaaacca

SEQ ID NO: 773 - RNA, 19 nt, synthetic construct
  source 1..19: mol_type = other RNA
atgtcaacaagaaaaaccc

SEQ ID NO: 774 - RNA, 19 nt, synthetic construct
  source 1..19: mol_type = other RNA
atgtcaacaagaaaaaccg

SEQ ID NO: 775 - RNA, 20 nt, synthetic construct
  source 1..20: mol_type = other RNA
atgtcaacaagaaaaaccct

SEQ ID NO: 776 - RNA, 20 nt, synthetic construct
  source 1..20: mol_type = other RNA
atgtcaacaagaaaaaccca

SEQ ID NO: 777 - RNA, 20 nt, synthetic construct
  source 1..20: mol_type = other RNA
atgtcaacaagaaaaacccc

SEQ ID NO: 778 - RNA, 20 nt, synthetic construct
  source 1..20: mol_type = other RNA
atgtcaacaagaaaaacccg

SEQ ID NO: 779 - RNA, 21 nt, synthetic construct
  source 1..21: mol_type = other RNA
atgtcaacaagaaaaaccctc

SEQ ID NO: 780 - RNA, 21 nt, synthetic construct
  source 1..21: mol_type = other RNA
atgtcaacaagaaaaaccctt

SEQ ID NO: 781 - RNA, 21 nt, synthetic construct
  source 1..21: mol_type = other RNA
atgtcaacaagaaaaacccta

SEQ ID NO: 782 - RNA, 22 nt, synthetic construct
  source 1..22: mol_type = other RNA
atgtcaacaagaaaaaccccgc

SEQ ID NO: 783 - RNA, 23 nt, synthetic construct
  source 1..23: mol_type = other RNA
atgtcaacaagaaaaaccccgcc

SEQ ID NO: 784 - RNA, 24 nt, synthetic construct
  source 1..24: mol_type = other RNA
atgtcaacaagaaaaaccccgcct

SEQ ID NO: 785 - RNA, 25 nt, synthetic construct
  source 1..25: mol_type = other RNA
atgtcaacaagaaaaaccccgcctg

SEQ ID NO: 786 - RNA, 26 nt, synthetic construct
  source 1..26: mol_type = other RNA
atgtcaacaagaaaaaccccgcctgt

SEQ ID NO: 787 - RNA, 32 nt, synthetic construct
  source 1..32: mol_type = other RNA
atgtcaacaagaaaaaccccgcctgtaacacg

SEQ ID NO: 788 - RNA, 23 nt, synthetic construct
  source 1..23: mol_type = other RNA
atgtcaacaagaaaaaccctgtt

SEQ ID NO: 789 - RNA, 23 nt, synthetic construct
  source 1..23: mol_type = other RNA
atgtcaacaagaaaaaccctgga

SEQ ID NO: 790 - RNA, 21 nt, synthetic construct
  source 1..21: mol_type = other RNA
atgtcaacaagaaaaaccctg

SEQ ID NO: 791 - RNA, 21 nt, synthetic construct
  source 1..21: mol_type = other RNA
atgtcaacaagaaaaaccctg

SEQ ID NO: 792 - RNA, 21 nt, synthetic construct
  source 1..21: mol_type = other RNA
atgtcaacaagaaaaaccctg

SEQ ID NO: 793 - RNA, 21 nt, synthetic construct
  source 1..21: mol_type = other RNA
atgtcaacaagaaaaaccctg

SEQ ID NO: 794 - RNA, 21 nt, synthetic construct
  source 1..21: mol_type = other RNA
acgtcaacaagaaaaaccctg

SEQ ID NO: 795 - RNA, 21 nt, synthetic construct
  source 1..21: mol_type = other RNA
atgtcaacaagaaaaaccctg

SEQ ID NO: 796 - RNA, 21 nt, synthetic construct
  source 1..21: mol_type = other RNA
cgggtttttcttgttgacaaa

SEQ ID NO: 797 - RNA, 21 nt, synthetic construct
  source 1..21: mol_type = other RNA
cgggtttttcttgttgacaat

SEQ ID NO: 798 - RNA, 21 nt, synthetic construct
  source 1..21: mol_type = other RNA
cgggtttttcttgttgacaac

SEQ ID NO: 799 - RNA, 21 nt, synthetic construct
  source 1..21: mol_type = other RNA
cgggtttttcttgttgacaag

SEQ ID NO: 800 - RNA, 17 nt, synthetic construct
  source 1..17: mol_type = other RNA
tttttcttgttgacaaa

SEQ ID NO: 801 - RNA, 18 nt, synthetic construct
  source 1..18: mol_type = other RNA
gtttttcttgttgacaaa

SEQ ID NO: 802 - RNA, 19 nt, synthetic construct
  source 1..19: mol_type = other RNA
agtttttcttgttgacaaa

SEQ ID NO: 803 - RNA, 19 nt, synthetic construct
  source 1..19: mol_type = other RNA
tgtttttcttgttgacaaa

SEQ ID NO: 804 - RNA, 19 nt, synthetic construct
  source 1..19: mol_type = other RNA
ggtttttcttgttgacaaa

SEQ ID NO: 805 - RNA, 19 nt, synthetic construct
  source 1..19: mol_type = other RNA
cgtttttcttgttgacaaa

SEQ ID NO: 806 - RNA, 20 nt, synthetic construct
  source 1..20: mol_type = other RNA
aggtttttcttgttgacaaa

SEQ ID NO: 807 - RNA, 20 nt, synthetic construct
  source 1..20: mol_type = other RNA
tggtttttcttgttgacaaa

SEQ ID NO: 808 - RNA, 20 nt, synthetic construct
  source 1..20: mol_type = other RNA
gggtttttcttgttgacaaa

SEQ ID NO: 809 - RNA, 20 nt, synthetic construct
  source 1..20: mol_type = other RNA
cggtttttcttgttgacaaa

SEQ ID NO: 810 - RNA, 21 nt, synthetic construct
  source 1..21: mol_type = other RNA
agggtttttcttgttgacaaa

SEQ ID NO: 811 - RNA, 21 nt, synthetic construct
  source 1..21: mol_type = other RNA
tgggtttttcttgttgacaaa

SEQ ID NO: 812 - RNA, 22 nt, synthetic construct
  source 1..22: mol_type = other RNA
cggggtttttcttgttgacaaa

SEQ ID NO: 813 - RNA, 23 nt, synthetic construct
  source 1..23: mol_type = other RNA
gcggggtttttcttgttgacaaa

SEQ ID NO: 814 - RNA, 24 nt, synthetic construct
  source 1..24: mol_type = other RNA
ggcggggtttttcttgttgacaaa

SEQ ID NO: 815 - RNA, 25 nt, synthetic construct
  source 1..25: mol_type = other RNA
aggcggggtttttcttgttgacaaa

SEQ ID NO: 816 - RNA, 26 nt, synthetic construct
  source 1..26: mol_type = other RNA
caggcggggtttttcttgttgacaaa

SEQ ID NO: 817 - RNA, 32 nt, synthetic construct; identical to SEQ ID NO: 695
  source 1..32: mol_type = other RNA

SEQ ID NO: 818 - RNA, 21 nt, synthetic construct
  source 1..21: mol_type = other RNA
cgggtttttcttgttgacaaa

SEQ ID NO: 819 - RNA, 21 nt, synthetic construct
  source 1..21: mol_type = other RNA
cgggtttttcttgttgacaaa

SEQ ID NO: 820 - RNA, 21 nt, synthetic construct
  source 1..21: mol_type = other RNA
cgggtttttcttgttgacaaa

SEQ ID NO: 821 - RNA, 21 nt, synthetic construct
  source 1..21: mol_type = other RNA
cgggtttttcttgttgacaaa

SEQ ID NO: 822 - RNA, 21 nt, synthetic construct
  source 1..21: mol_type = other RNA
cgggtttttcttgttgacaaa

SEQ ID NO: 823 - RNA, 21 nt, synthetic construct
  source 1..21: mol_type = other RNA
cgggtttttcttgttaacaaa

SEQ ID NO: 824 - RNA, 21 nt, synthetic construct
  source 1..21: mol_type = other RNA
cgggtttttcttgttgacaga

SEQ ID NO: 825 - RNA, 21 nt, synthetic construct
  source 1..21: mol_type = other RNA
cgggtttttcttgttgacaaa

SEQ ID NO: 826 - RNA, 21 nt, synthetic construct
  source 1..21: mol_type = other RNA
cagggtttttcttgttgacat

SEQ ID NO: 827 - RNA, 21 nt, synthetic construct
  source 1..21: mol_type = other RNA
cagggtttttcttgttgacaa

SEQ ID NO: 828 - RNA, 21 nt, synthetic construct
  source 1..21: mol_type = other RNA
cagggtttttcttgttgacac

SEQ ID NO: 829 - RNA, 21 nt, synthetic construct
  source 1..21: mol_type = other RNA
cagggtttttcttgttgacag

SEQ ID NO: 830 - RNA, 17 nt, synthetic construct
  source 1..17: mol_type = other RNA
gtttttcttgttgacat

SEQ ID NO: 831 - RNA, 18 nt, synthetic construct
  source 1..18: mol_type = other RNA
ggtttttcttgttgacat

SEQ ID NO: 832 - RNA, 19 nt, synthetic construct
  source 1..19: mol_type = other RNA
aggtttttcttgttgacat

SEQ ID NO: 833 - RNA, 19 nt, synthetic construct
  source 1..19: mol_type = other RNA
tggtttttcttgttgacat

SEQ ID NO: 834 - RNA, 19 nt, synthetic construct
  source 1..19: mol_type = other RNA
gggtttttcttgttgacat

SEQ ID NO: 835 - RNA, 19 nt, synthetic construct
  source 1..19: mol_type = other RNA
cggtttttcttgttgacat

SEQ ID NO: 836 - RNA, 20 nt, synthetic construct
  source 1..20: mol_type = other RNA
agggtttttcttgttgacat

SEQ ID NO: 837 - RNA, 20 nt, synthetic construct
  source 1..20: mol_type = other RNA
tgggtttttcttgttgacat

SEQ ID NO: 838 - RNA, 20 nt, synthetic construct
  source 1..20: mol_type = other RNA
ggggtttttcttgttgacat

SEQ ID NO: 839 - RNA, 20 nt, synthetic construct
  source 1..20: mol_type = other RNA
cgggtttttcttgttgacat

SEQ ID NO: 840 - RNA, 21 nt, synthetic construct
  source 1..21: mol_type = other RNA
gagggtttttcttgttgacat

SEQ ID NO: 841 - RNA, 21 nt, synthetic construct
  source 1..21: mol_type = other RNA
aagggtttttcttgttgacat

SEQ ID NO: 842 - RNA, 21 nt, synthetic construct
  source 1..21: mol_type = other RNA
tagggtttttcttgttgacat

SEQ ID NO: 843 - RNA, 22 nt, synthetic construct
  source 1..22: mol_type = other RNA
gcggggtttttcttgttgacat

SEQ ID NO: 844 - RNA, 23 nt, synthetic construct
  source 1..23: mol_type = other RNA
ggcggggtttttcttgttgacat

SEQ ID NO: 845 - RNA, 24 nt, synthetic construct
  source 1..24: mol_type = other RNA
aggcggggtttttcttgttgacat

SEQ ID NO: 846 - RNA, 25 nt, synthetic construct
  source 1..25: mol_type = other RNA
caggcggggtttttcttgttgacat

SEQ ID NO: 847 - RNA, 26 nt, synthetic construct
  source 1..26: mol_type = other RNA
acaggcggggtttttcttgttgacat

SEQ ID NO: 848 - RNA, 32 nt, synthetic construct; identical to SEQ ID NO: 726
  source 1..32: mol_type = other RNA

SEQ ID NO: 849 - RNA, 21 nt, synthetic construct
  source 1..21: mol_type = other RNA
cagggtttttcttgttgacat

SEQ ID NO: 850 - RNA, 21 nt, synthetic construct
  source 1..21: mol_type = other RNA
cagggtttttcttgttgacat

SEQ ID NO: 851 - RNA, 21 nt, synthetic construct
  source 1..21: mol_type = other RNA
cagggtttttcttgttgacat

SEQ ID NO: 852 - RNA, 21 nt, synthetic construct
  source 1..21: mol_type = other RNA
cagggtttttcttgttgacat

SEQ ID NO: 853 - RNA, 21 nt, synthetic construct
  source 1..21: mol_type = other RNA
cagggtttttcttgttgacat

SEQ ID NO: 854 - RNA, 21 nt, synthetic construct
  source 1..21: mol_type = other RNA
cagggtttttcttgtcgacat

SEQ ID NO: 855 - RNA, 21 nt, synthetic construct
  source 1..21: mol_type = other RNA
cagggtttttcttgttgacgt

SEQ ID NO: 856 - RNA, 21 nt, synthetic construct
  source 1..21: mol_type = other RNA
cagggtttttcttgttgacat

SEQ ID NO: 857 - RNA, 21 nt, synthetic construct
  source 1..21: mol_type = other RNA
tttgtcaacaagaaaaacccg

SEQ ID NO: 858 - RNA, 21 nt, synthetic construct
  source 1..21: mol_type = other RNA
attgtcaacaagaaaaacccg

SEQ ID NO: 859 - RNA, 21 nt, synthetic construct
  source 1..21: mol_type = other RNA
gttgtcaacaagaaaaacccg

SEQ ID NO: 860 - RNA, 21 nt, synthetic construct
  source 1..21: mol_type = other RNA
cttgtcaacaagaaaaacccg

SEQ ID NO: 861 - RNA, 17 nt, synthetic construct
  source 1..17: mol_type = other RNA
tttgtcaacaagaaaaa

SEQ ID NO: 862 - RNA, 18 nt, synthetic construct
  source 1..18: mol_type = other RNA
tttgtcaacaagaaaaac

SEQ ID NO: 863 - RNA, 19 nt, synthetic construct
  source 1..19: mol_type = other RNA
tttgtcaacaagaaaaact

SEQ ID NO: 864 - RNA, 19 nt, synthetic construct
  source 1..19: mol_type = other RNA
tttgtcaacaagaaaaaca

SEQ ID NO: 865 - RNA, 19 nt, synthetic construct
  source 1..19: mol_type = other RNA
tttgtcaacaagaaaaacc

SEQ ID NO: 866 - RNA, 19 nt, synthetic construct
  source 1..19: mol_type = other RNA
tttgtcaacaagaaaaacg

SEQ ID NO: 867 - RNA, 20 nt, synthetic construct
  source 1..20: mol_type = other RNA
tttgtcaacaagaaaaacct

SEQ ID NO: 868 - RNA, 20 nt, synthetic construct
  source 1..20: mol_type = other RNA
tttgtcaacaagaaaaacca

SEQ ID NO: 869 - RNA, 20 nt, synthetic construct
  source 1..20: mol_type = other RNA
tttgtcaacaagaaaaaccc

SEQ ID NO: 870 - RNA, 20 nt, synthetic construct
  source 1..20: mol_type = other RNA
tttgtcaacaagaaaaaccg

SEQ ID NO: 871 - RNA, 21 nt, synthetic construct
  source 1..21: mol_type = other RNA
tttgtcaacaagaaaaaccct

SEQ ID NO: 872 - RNA, 21 nt, synthetic construct
  source 1..21: mol_type = other RNA
tttgtcaacaagaaaaaccca

SEQ ID NO: 873 - RNA, 22 nt, synthetic construct
  source 1..22: mol_type = other RNA
tttgtcaacaagaaaaaccccg

SEQ ID NO: 874 - RNA, 23 nt, synthetic construct
  source 1..23: mol_type = other RNA
tttgtcaacaagaaaaaccccgc

SEQ ID NO: 875 - RNA, 24 nt, synthetic construct
  source 1..24: mol_type = other RNA
tttgtcaacaagaaaaaccccgcc

SEQ ID NO: 876 - RNA, 25 nt, synthetic construct
  source 1..25: mol_type = other RNA
tttgtcaacaagaaaaaccccgcct

SEQ ID NO: 877 - RNA, 26 nt, synthetic construct
  source 1..26: mol_type = other RNA
tttgtcaacaagaaaaaccccgcctg

SEQ ID NO: 878 - RNA, 32 nt, synthetic construct; identical to SEQ ID NO: 756
  source 1..32: mol_type = other RNA

SEQ ID NO: 879 - RNA, 23 nt, synthetic construct
  source 1..23: mol_type = other RNA
tttgtcaacaagaaaaacccgtt

SEQ ID NO: 880 - RNA, 23 nt, synthetic construct
  source 1..23: mol_type = other RNA
tttgtcaacaagaaaaacccgga

SEQ ID NO: 881 - RNA, 21 nt, synthetic construct
  source 1..21: mol_type = other RNA
tttgtcaacaagaaaaacccg

SEQ ID NO: 882 - RNA, 21 nt, synthetic construct
  source 1..21: mol_type = other RNA
tttgtcaacaagaaaaacccg

SEQ ID NO: 883 - RNA, 21 nt, synthetic construct
  source 1..21: mol_type = other RNA
tttgtcaacaagaaaaacccg

SEQ ID NO: 884 - RNA, 21 nt, synthetic construct
  source 1..21: mol_type = other RNA
tttgtcaacaagaaaaacccg

SEQ ID NO: 885 - RNA, 21 nt, synthetic construct
  source 1..21: mol_type = other RNA
tctgtcaacaagaaaaacccg

SEQ ID NO: 886 - RNA, 21 nt, synthetic construct
  source 1..21: mol_type = other RNA
tttgtcaacaagaaaaacccg

SEQ ID NO: 887 - RNA, 21 nt, synthetic construct
  source 1..21: mol_type = other RNA
atgtcaacaagaaaaaccctg

SEQ ID NO: 888 - RNA, 21 nt, synthetic construct
  source 1..21: mol_type = other RNA
ttgtcaacaagaaaaaccctg

SEQ ID NO: 889 - RNA, 21 nt, synthetic construct
  source 1..21: mol_type = other RNA
gtgtcaacaagaaaaaccctg

SEQ ID NO: 890 - RNA, 21 nt, synthetic construct
  source 1..21: mol_type = other RNA
ctgtcaacaagaaaaaccctg

SEQ ID NO: 891 - RNA, 17 nt, synthetic construct
  source 1..17: mol_type = other RNA
atgtcaacaagaaaaac

SEQ ID NO: 892 - RNA, 18 nt, synthetic construct
  source 1..18: mol_type = other RNA
atgtcaacaagaaaaacc

SEQ ID NO: 893 - RNA, 19 nt, synthetic construct
  source 1..19: mol_type = other RNA
atgtcaacaagaaaaacct

SEQ ID NO: 894 - RNA, 19 nt, synthetic construct
  source 1..19: mol_type = other RNA
atgtcaacaagaaaaacca

SEQ ID NO: 895 - RNA, 19 nt, synthetic construct
  source 1..19: mol_type = other RNA
atgtcaacaagaaaaaccc

SEQ ID NO: 896 - RNA, 19 nt, synthetic construct
  source 1..19: mol_type = other RNA
atgtcaacaagaaaaaccg

SEQ ID NO: 897 - RNA, 20 nt, synthetic construct
  source 1..20: mol_type = other RNA
atgtcaacaagaaaaaccct

SEQ ID NO: 898 - RNA, 20 nt, synthetic construct
  source 1..20: mol_type = other RNA
atgtcaacaagaaaaaccca

SEQ ID NO: 899 - RNA, 20 nt, synthetic construct
  source 1..20: mol_type = other RNA
atgtcaacaagaaaaacccc

SEQ ID NO: 900 - RNA, 20 nt, synthetic construct
  source 1..20: mol_type = other RNA
atgtcaacaagaaaaacccg

SEQ ID NO: 901 - RNA, 21 nt, synthetic construct
  source 1..21: mol_type = other RNA
atgtcaacaagaaaaaccctc

SEQ ID NO: 902 - RNA, 21 nt, synthetic construct
  source 1..21: mol_type = other RNA
atgtcaacaagaaaaaccctt

SEQ ID NO: 903 - RNA, 21 nt, synthetic construct
  source 1..21: mol_type = other RNA
atgtcaacaagaaaaacccta

SEQ ID NO: 904 - RNA, 22 nt, synthetic construct
  source 1..22: mol_type = other RNA
atgtcaacaagaaaaaccccgc

SEQ ID NO: 905 - RNA, 23 nt, synthetic construct
  source 1..23: mol_type = other RNA
atgtcaacaagaaaaaccccgcc

SEQ ID NO: 906 - RNA, 24 nt, synthetic construct
  source 1..24: mol_type = other RNA
atgtcaacaagaaaaaccccgcct

SEQ ID NO: 907 - RNA, 25 nt, synthetic construct
  source 1..25: mol_type = other RNA
atgtcaacaagaaaaaccccgcctg

SEQ ID NO: 908 - RNA, 26 nt, synthetic construct
  source 1..26: mol_type = other RNA
atgtcaacaagaaaaaccccgcctgt

SEQ ID NO: 909 - RNA, 32 nt, synthetic construct; identical to SEQ ID NO: 787
  source 1..32: mol_type = other RNA

SEQ ID NO: 910 - RNA, 23 nt, synthetic construct
  source 1..23: mol_type = other RNA
atgtcaacaagaaaaaccctgtt

SEQ ID NO: 911 - RNA, 23 nt, synthetic construct
  source 1..23: mol_type = other RNA
atgtcaacaagaaaaaccctgga

SEQ ID NO: 912 - RNA, 21 nt, synthetic construct
  source 1..21: mol_type = other RNA
atgtcaacaagaaaaaccctg

SEQ ID NO: 913 - RNA, 21 nt, synthetic construct
  source 1..21: mol_type = other RNA
atgtcaacaagaaaaaccctg

SEQ ID NO: 914 - RNA, 21 nt, synthetic construct
  source 1..21: mol_type = other RNA
atgtcaacaagaaaaaccctg

SEQ ID NO: 915 - RNA, 21 nt, synthetic construct
  source 1..21: mol_type = other RNA
atgtcaacaagaaaaaccctg

SEQ ID NO: 916 - RNA, 21 nt, synthetic construct
  source 1..21: mol_type = other RNA
acgtcaacaagaaaaaccctg

SEQ ID NO: 917 - RNA, 21 nt, synthetic construct
  source 1..21: mol_type = other RNA
atgtcaacaagaaaaaccctg

SEQ ID NO: 918 - RNA, 21 nt, synthetic construct
  source 1..21: mol_type = other RNA
cagggtttttcttgttgacat

SEQ ID NO: 919 - RNA, 21 nt, synthetic construct
  source 1..21: mol_type = other RNA
cgggtttttcttgttgacaaa

SEQ ID NO: 920 - RNA, 21 nt, synthetic construct
  source 1..21: mol_type = other RNA
gttactagtgccatttgttca

SEQ ID NO: 921 - RNA, 21 nt, synthetic construct
  source 1..21: mol_type = other RNA
ggttaccaattttcttttgta

SEQ ID NO: 922 - RNA, 21 nt, synthetic construct
  source 1..21: mol_type = other RNA
atgtcaacaagaaaaaccctg

SEQ ID NO: 923 - RNA, 21 nt, synthetic construct
  source 1..21: mol_type = other RNA
tttgtcaacaagaaaaacccg

SEQ ID NO: 924 - RNA, 21 nt, synthetic construct
  source 1..21: mol_type = other RNA
tgaacaaatggcactagtaac

SEQ ID NO: 925 - RNA, 21 nt, synthetic construct
  source 1..21: mol_type = other RNA
tacaaaagaaaattggtaacc